European Patent Specification EP 3 870 690 B1, published June 24, 2026. Title: Sporeforming probiotic strains, methods and uses thereof. Applicant: CIIMAR - CENTRO INTERDISCIPLINAR DE INVESTIGAÇÃO MARINHA E AMBIENTAL Universidade do Porto. The sequence listing filed with the application follows.

SEQUENCE LISTING (207 sequences)

SEQ ID NO: 1 - protein, 202 aa, Bacillus subtilis
  >ABP10118
MNLTGESKNFDDYLLELNEVDYSNPIICALANELFNPLQTEIEKVKIAYEFVRDEISHTWDTQSKRVTCNASEVLSFKEGICYAKSNLLAALLRSEGIPTGFCYQRLMLFNTPDKGYCIHALNAVFFHSLNKWIRLDSRGNKIGIDAQFSLDKERLAFPIRQEFDEIDYPLIYVRPHPKTIAVLKEHKDAIEMYKYHLPERI

SEQ ID NO: 2 - protein, 215 aa, Bacillus subtilis
  >ABP10119
MIWLVGLDWSIQWGTVFTVAGTLTAAFLGQVFSHRYSQKREEIKQKKESFQNLYSPVVFKILNYLELEREKQNIMFIKGLDETEFTERYQDDELYNPSIEFKEILEIVGLNLKYGSLELIREYQETLSIAKRMEAFEGHCGTHLYFCGVFISDYINLSKDLGVYSQTMETSTEGSLLLSRLETLIPQLVVLECLWNFYLGFFMQYLVLIKKINIL

SEQ ID NO: 3 - protein, 286 aa, Bacillus subtilis
  >ABP10120
MELKNKIKRVAIYLRKSRNKEGEETEETLAKHRKRLLDIAHKNNWQYEIFQEVGSSMDEMRPECQRMINKLTDGIFDAVLSVNLARVTRDDAETPKFMNLLRQDDILFVTDSERVYDLEVQEDWQALKFTGFVNNWEYENIKAQLRKGKKDSAKMGRWSNGKPNYGYIYNRLERKLEIDEEKAKAVKLAFQMTIDGIGADNIAVKLNKLGYRTNKGKFFHGQSIVRMIRSEIYKGWIVANRLKGRNKTNGKIRPQDQWIVVKDAVKPCIIDEDTWDKANKAGHLIK

SEQ ID NO: 4 - protein, 153 aa, Bacillus subtilis
  ABP10121
MYSYKLIDNEKVREKLEELIDEKREIHLKLTDNHLDKHLGITYDLLDVNDDGSYSGFFRTTPYIRRSDLILPGESIGIKLPSYFLIMINYLSRLEEQDCFPELELKITYNDTNFKTWETKFIIKVDQISKIEISSFYKLQTSLVYEFISKNKK

SEQ ID NO: 5 - protein, 604 aa, Bacillus subtilis
  >ABP10181
MAVVTTIKHPMISGYVKGFVDKYEISRRKAKNEHNIFEMFINDLILSSYNNDPNASYEDMETGTAFGIDGVAIFINDKLVEGVEDVDYICNSTRKIEVKFLFTQTKTSEKFDRSEVRDFLQGVNRFFNFEFCEITELKNSWETAKYIYDLSTKFKNDPALKMYYTALAPKKISVKDEDIDLHLKSEILTGLEVLKQRYIFDEDNISLNFIGLKEIRELHQKENNLTEIKFNLDKQPVPYPKDSTGIIKSAYFGLIKLEDLLDILSEAVDGERILRKGIFEDNIRDYLGANEKFDVNLDMKNGLTGTNAHLFGLLNNGITIIADQVHIISTEASLVNYQIVNGCQTSNVIFESLKDIIEKNIYIPIRLIGTEDEDTKNAIIKATNSQTALKPEQLLALRDEQKSLEEYYRAKRNQNKFLLYYERRTEQYRNEDIQKTKIINIPFQIKATSAMFLDLPHEVSGQYGKVEQKTRGKLFTDSSLLNPYYVSGLTWYRVEAFIRNNEEGKKHRRARWHIMMVIKYLISDLKNPSKIIDKNAEKISEKVEKVMLNDAKSLEIIENALSLIKEFIINEGILDISEDRKFFERKETTTGLIEMLKNRLKTLS

SEQ ID NO: 6 - protein, 851 aa, Bacillus subtilis
  >ABP10182
MEHSNKLNIVYKSIQQMKESYGKLLKVEFHIHTPASHDYRLLPGKLFKNMKLTEVFDVALNEGLYSKEFLERIQKEDFAIFEKQVIEDINRDFHVSFSNFKEILGYQLIAHSLYKNNIHAAVISDHNTINGFKKLQAVLVDYYKSRIKGNTQRKSIKLFLGIEISCSDYYHLVGIFDEHKYTDLKNFVSKYIHSEEEGTYISCLDMVNRITENGGIPYIAHINTSDFLGTNLYKRSLFGFSGLKILGLTNIDSKERISNRIKKYQESSKGDFCFIHEGDSHELNQLGKKNTWIKFNNLSFKSLKKAFKNYQFCIYIDKPIYNDRFLKGIYIEPGEKGFLGDKEQPEKPFIVDFSRDLNCIIGGRGVGKSTILSILETAFTLEVTNINQLEYISRHNLIYIVFNYKNMDYILNFIPQITESGYSGNNYFLRKAFSETTETESGTRRLSQNWINLYRVSQVESSNGYKFQELNYNETTTIIESVYKKSYSINNIVELSNTGRISEFIRDIVLNGERLNGSKIVLSKLNKLHKNNYRKYLRENIQSVLVNIKKREENVKMAIEEFNRLNNKLIQIVYSPKLKDPTFYLKELELRYDPIFDREKGKRVLNTYLTWDDIDEFVYEATKKFGYLEFLELILNKEHKQIENELSLNNFISGTITGEYENVSIKNMVRVYNKIEERIFRNIEKVTNSFKLLFEIIDEFSLKFNINSKETIRTEKVVMKDIDELSLGQKVVAILTLIFNYGEHSVDSTPLVIDQPEDNLDNLYIYQNLVKSLRKIKNKRQVIIATHSATIVTNADAEQVIILESDNKRGWLSKKGYPDDEVVLKHIVSILEGGRESFIHKKETYMTVLDI

SEQ ID NO: 7 - protein, 316 aa, Bacillus subtilis
  >ABP10654
MTQSPIFLTPVFKEKIWGGTALRDRFGYSIPSETTGECWAISAHPKGPSTVANGPYKGKTLIELWEEHREVFGGVEGDRFPLLTKLLDVKEDTSIKVHPDDYYAGENEEGELGKTECWYIIDCKENAEIIYGHTARSKTELVTMINSGDWEGLLRRIKIKPGDFYYVPSGTLHALCKGALVLETQQNSDATYRVYDYDRLDSNGSPRELHFAKAVNAATVPHVDGYIDESTESRKGITIKTFVQGEYFSVYKWDINGEAEMAQDESFLICSVIEGSGLLMYEDKTCLLKKGDHFILPAQMPDFTIKGTCTLIVSHI

SEQ ID NO: 8 - protein, 880 aa, Bacillus subtilis
  >ABP10655
MKKRLIAPMLLSAASLAFFAMSGSAQAAAYTDYSLYKVEPSNTFSTESQASQAVAKLEKDTGWDASYQASGTTTTYQISASGIHSESEAKAILSGLAKQTSITGTSSPVGSKQPYVTISSGAISGEKQANTILAKLKQETGVAGAVKAYGAAQPYMNVMTSDIADETKVKALIQSLAKQTGIKSSYQPITHTVSVTTIQSGTIVGDSRAAQIKNAFQKESGLQASLKETVKGQAYYTFTTAAISGEANAKTLLQQLKQSTGITGSYKSINQKTTVESYNVQSAYFKGLNTVKDAISQIKKNTGVSGSYQQVGKSTSYTVNMKGITKQQLQKIDTFFKKKKWHYTSSSVKKTTTSAAYQITTAKILGEQQANKAAAFFAQKKVKATKTTAGTTAENQYQLISEETSDQSKVTKGLNILKKNQLSASAKSVKKQIADTFKITTESLLDQTKVNQALTFFKSNHISAASQKTGQTAASSYQITTEAIISQEEIDRVLTFFKQNKIAVTTSKTGQTAYTQYKIVTAQLSSKTALNNGLTYLKSQGLTPSYTTKSNTLYKISVNEQFTGNDTAAAASSKLKQLYGWASSIVKVKNGPQIMKTNYNLSLRDMVQKQMTVSPQTDGAAYVSLTYINTATSTVTADALNIRSTPEVSPTNVIGQFKKGDKVKIIGQTNGWAKINLGWRNASSDEVVQYVDPNNFSRDSKYYFQFLKLSQTAGLNATEVNQKVLAGKGILTGKAKAFIDAANKYGINELYLISHALLETGNGTSDLANGLTYNGKTVYNMYGIGAYDSNPNYYGAKYAYEQGWFTPEAAIIGGAKFIGSSYIHNTAYNQDTLYKMRWSATATHQYATDIGWAYKQVNRMYSLYSLLDGYTLYFDVPEFK

SEQ ID NO: 9 - protein, 37 aa, Bacillus subtilis
  >ABP10656
MYYLEIMIKMLKEIRKEPKKFDIIFVSSPPFLLLLSG

SEQ ID NO: 10 - protein, 254 aa, Bacillus subtilis
  >ABP10657
MKGVKVFHHPIIVESFRILEKLLYKKADHIVINSEGFLHYLNEHSPLVKEKVTFIPNSAREKELLISSNDAKTALKIIYVGNIGLAQNVHIIRNLAEKLHEHQIEFLIVGYGVEKKELLNYIREKNLMNVKIVNPMTRKECLELMSGCDIGIVTLKDSTVFETVLPGRIIDYITCGIPIVGSIAGYSKTIIEQEGVGLVTSNSSSEEMLANIMKIYNDPGLLKKMQKNCHKLIRENFMWETNIEKLINVIEDTR

SEQ ID NO: 11 - protein, 422 aa, Bacillus subtilis
  >ABP10658
MRKKVCMFVWNHFTNDARVLRECTALSDKYYDVDLICIHDPNNPDLDLIQKYNDHFTVYRVKRSPLLFYIQFIYKLFKNKWSILFFLLIWICLLRMFPLLTIGFSLFAVIVLKTKLKTMLVRGSIIMRMILKGYSKKYDIYHSNDLNTLPQGFICSKFRFKKRKLIYDSHEVQTSRTGYDSPFYSKMEAYLIRKIDIMIVENHTRAAYNKELYGFYPKVLHNYPFLLEETKEQIDIHHMLGLPKNEKILLYQGGIQVGRGLDKLIKAMPFINEGTLLFIGDGRIKKDLENMVNNMELQHRVRFLPKVPLSELPKYTRSAYLGFQVLNNVCFNHYSASSNKLFEYIMAGVPVIGCDFPEIKKVIQGEKVGLVVDSHDHLSIAKGVNTLLENADLHYEFHKNCDKAKRKYNWETEKSQLLSLYN

SEQ ID NO: 12 - protein, 74 aa, Bacillus subtilis
  >ABP10659
MQIKKNQKNQELADKYNDLKIKYHKSLEVQEDLITLCQELIREKEYIEARYNNLKESKLGRLTVWMWKRRRRNK

SEQ ID NO: 13 - protein, 771 aa, Bacillus subtilis
  >ABP10660
MKQSKDIKTLLSKQLEKVRREKEILIGLKEKEVSITGFDDFFFDTPMRILAEYNKQTLEVDAEKVYLSLFERTTNFSIPSNKEIYKLTGDRIIIDPFITLSGSVKGQIYIAFYKNNELYSTKIFEAPFDKISADVPENTTSYRFALRLEGKGYLQLNKLKIKQVFKEQIASKNIGVNRSITISKASKIQQFIDSIEAETQNYKNEKKELRIAAILDEFSYECFKHDAEILRLSNTDWDNEILEFNPHFVFVESCWQGNQGHWQYEVANLHKNKHRTALKKLTEYCKSKNIKTVFWDKEGYENFEFFKTAASYFDYVMTADENTVKKFKETSSINNVGILPFAAQPRIHNPINKNLHHLGGIAFAGSYYNNKHESRKRDIEEIIKPALDFGIDIYDRYYNVPAAKKVNNTWPEEYQRHIVGSLNYSQMNVAYKNYNMFVNVNSVQNSKHMFARRVFELLASKTMVISGPSKGVQEYFGDLVPVACSKEETVNILKTFLYNPVYREMYEKKGHRLVLNSHTYKNRLQEICDHIGIDINLLEKPRISIISSTQRTEYMENLYNNARHQTYQNLELIIILNKNSMDAEEWKQKFSSLHFPVTILQVDENVSLGHCLNKAVQRSTGEIIAKFDDDDYYAPHYLEDMLHSMEYSGADIVGKSAHYVYLEERELLILKTVGSGAERYSDFISGATLVFKKEVFVSLGGFSDKNRGEDSDFLKRAKENGNIIYSNDSWNFCLVRRANRNSHTWNITADDLLRNSTVHSMCKDYKKPITI

SEQ ID NO: 14 - protein, 425 aa, Bacillus subtilis
  >ABP10661
MKVCVIGLGYIGLPTSVMFAKYGVDVIGVDVQPHVVDSLNNGEAHLEEPGLQEFLDEALANGNFKAQLVPEPADAFIIAVPTPNNINDNMSCDLTYVLQAVDNIIPYIRKGSTIIVESTIAPRSIEDYVQPLLEQNGFTIGEDIYLVHCPERVMPGNIFHELANNMRIVGGITPSCSEAGEKVYRTFVKSKIVKTDAKTAEMSKLMENTYRDVNIALANELTKICNDLHINALDVIEMANMHPRVNIHSPGPGVGGHCLAVDPYFIVAKAPETADLISRSRSINSSMPIYIVEKVREIMEMVNGRTITIGGLAYKGDIDDLRESPALEILEMLKSEKKYEVRAYDPYVNHSENAQNLTEALGGSDLFLILTDHSLFKTINDEDTNRMSNKVIFDTRNIVRNVPEDCECINLGSIHNFLNNAVLNV

SEQ ID NO: 15 - protein, 710 aa, Bacillus subtilis
  ABP10662
MRKYLCLFSFVILFFLTLSFYGERVLAYTDTSTYKVTIKDEFTSEDKVKGISNKINNETGWDANYKLTGNTTRAFKIITGGFYGEDKVKDVLNDFEQNTGINGSYSENGNVQTIYQITTGGFTGESKVKQVLDILQSQTGVKGTYTSTGEKQYYYRIVSGGFQSEQRIKEVLSKFENETSIKGSYEPIGNSKITYTVLSGGFSTEDNVKKAAAETKSQTGIEASYEKIPDSESYRLVISNITESELTGIESFFGKKNWWYVKKEVKNQSYRLISEPILDDQIIDKGLSFFESNKWWASKQKTDQLGENKFRITTEKISDETKLLKALNFFESNKWWAVSQKTTIKGYRITSEVINSEAVLNKGLDFFKSKNLWATYSNLSKDTYIINLNEEFTGIENATSAVNKLSNVYGLNAEVVKIKDGPQIMNTNYNLTLSDMISKQMNANPQTDSAAYVSLSYINTSTSTVTADYLNVRSTPEVKSDNIIGQVQKSDKVTIISKEGNWAKINMGWRKASREEVTYYINPENFSISSKYYFQFLKLSQYAGLTATEVNNKILKGKGILEGKGESFIKAAESNNINELYLIAHSLLETGNGSSELANGVMYNGKKVYNMYGIGAYDGDAVTKGAQYAYNQGWFTPEAAILGGAKFIGSSYIHNATYHQDTLYKMRWEPTVSHQYATDIGWAYKQVNRMYSLYTLLDNYTLYYDIPKYK

SEQ ID NO: 16 - protein, 280 aa, Bacillus subtilis
  >ABP10663
MEINQLRKETIKFIDLKEYKIRIEEPYLLCVTTEDGVPFEFLINIRLNQNKLLILSSGAYDNVKLKPPIFQRYTWMTEFNHSVVYFNDPTLYINQKLSIGWGQGTKNHFYLATITNVIRELAYKIKVNTKDIFFYGSSAGGFMSLILASFLRANAIVNNPQTDVCTFYQSHVDRLFETLYPNEDKHEVIKQFRYRLNVCAFFQKLKQVPKIFYYQNYACSFDVETQLIPFLNSIKSEKTLAHLTADKEIELHLYYDAELGHNPLNKQKTMEIIHKAMFGS

SEQ ID NO: 17 - protein, 623 aa, Bacillus subtilis
  ABP10664
MRYKVKLARKIKNRLFRSKKKTQKENAAVIVHPADNRVFSLFDKTKRIEENQQVPVRKISEFSWNGSILKIAGYMYIKGLPLQKEDQVRKRLLLVNNGVLFTAVSLRDVPVDKLSIDTSNVPGAYKWAGFSQQINFSKLMNDKPLPQGEYKLFLEIEAVDDQNVKHQEVHTVGNVSNFLSNDVYATKMEFHSAKKLMKFNLIVNYDEGEKTINLSCNKLQEIDPSLLELDTGKEANRFLRKLNTSLFHFAYDVFRLLPIKSNKIVFASDSRLDMTGNFEFVYEELLKREENFDFKFFLKSSIRDRKSLSELMSMAYHFATSKIIFIDDFYPIIYPLKIRKNADLVQLWHAVGAFKTFGYSRIGLPGGPSPHSKNHRNYTKVIVSSENIRKHYAEGFGVDIENVIATGVPRTDFFFDEAKKAFVKERLYTEYPFLKDKKVILFAPTFRGNGQQSAHYPFEVLDFDRLYRELKDEYIFLFKIHPFVRNDANIPYQYSDFFYDFSSFREINELLLVTDILITDYSSVCFEYALLNKPMIFFSYDVDDYIRKRDFYYDYFDFIPGPLAKTSEQMISIIKEEKYNFEQIDSFVHYFFDDLDGKASERVVDQIVFPQEEEPSEDKVLKR

SEQ ID NO: 18 - protein, 389 aa, Bacillus subtilis
  >ABP10665
MKTFLTRIVKGVFGTAYKLLSALLPVQHNKIVIASYREDHLSDNFKGVYEKLKQDPSLRITLLFRKMDKGLIGRVAYLLHLFSSLYHLATCRVLLLDDYYFPLYVVPKRKETVAIQLWHACGAFKKFGYSIVNKPFGPSSDYLKIVPVHSNYDYAIVSAPAAVPHFAEAFQMEQKQILPLGIPRTDYFYHKEHIRTVLDEFHRVYPELKHKKKLLYAPTFRGSGHHQEGDAIPLDLLQLKSALSHKDYVVILHLHPYMRKHAHTEEDDFVLDLTDSYSLYDLMAISDGLITDYSSVIFEYSLLKRPMYFYCPDLEDYLEERDFYYPFESFVPGPISKDVPSLVHDIESDHEADTKRIEDFSQAFITHQDGKSSGRVADFISSFLTSGAD

SEQ ID NO: 19 - protein, 163 aa, Bacillus subtilis
  >ABP10666
MTLLLKKKYPDSKVFIFGKTPYKLDHFSFVDAAYQINDIPEDVRIDHAFECVGGRGSESAIEQIIAHVHPEACVALLGVSEYPVEIETRMVLEKGITLIGSSRSGREDFARTVDFLAQYPEVVDYLETLVGGRFPVRSIEEITNAFEADLTSSWGKTVIEWEI

SEQ ID NO: 20 - protein, 178 aa, Bacillus subtilis
  >ABP10667
MINQTYRLVSARQFEVTYKDKVVHSDKVVVRPTHLSICAADQRYYTGSRGKEAMDKKLPMALIHEGIGKVMFDPTGTFKVGTRVVMVPNTPVEEHEVIAENYLRSSRFRSSGYDGFMQDYMFMAPDRLVELPDSINPHVAAFTELITIAVHALSRFERMAHKKRDTFGVWGTEISDLS

SEQ ID NO: 21 - protein, 237 aa, Bacillus subtilis
  >ABP10668
MIYAEILAGGKGSRMGNVNMPKQFLPLNKRPIIIHTIEKFLLNDRFDKILIVSPKEWINHTKDILKKFIGQDDRLIVVEGGSDRNESIMSGIRYIEKEFGIQDDDVIITHDSVRPFLTHRIIDENIDAVLQYGAVDTVISAIDTIIASEDQEFISDIPVRDNMYQGQTPQSFRISKLVELYNKLSDEQKAVLTDACKICSLAGEKVKLVRGEVFNIKVTTPYDLKVANAILQERISQ

SEQ ID NO: 22 - protein, 355 aa, Bacillus subtilis
  >ABP10669
MTLLVSFPDNARAILKEYQMGHYSFPIHVLLTQHAKSLETEFPELTVSVINEKHPLHIYKAVFSMLSSKAVIVDNYFVLTTVLTCRPDIECIQVWHANGAFKRFGLKDINTQNRSRADVRRFRKVYASFDRIVVGSEHMADIFKEFFDIKGDKFLRFGVPLTDAYYEVQENSNDLKNKYHLPADKKIILYAPTFRDHQFESFSLPFSEKQLQHDLKGEYLLAVKLHPVMKQSAELPGDSAWIKDVSDLPLADLLKMSDLLISDYSSVPFEFALLDKPILFYTYDMEAYNRTRGLIRNYSEVIPGVPCCDSRALLDQLKVMDNLQSEFERFSREWNLYSRGNASKQLLSYINEKSI

SEQ ID NO: 23 - protein, 65 aa, Bacillus subtilis
  >ABP10670
MTSRFDPKQQCADDFDEQIVKKRKPGFQSVISSKRLPRIVGRHSERFMHFITYHSSFKAHYRWRD

SEQ ID NO: 24 - protein, 257 aa, Bacillus subtilis
  >ABP10671
MQTKPINQLDFVDGELTSFVSHLETSFLDQNKGAFIVTANPEIGFEAMQNPRYEAVLSSADFILPDGIGVVLVSKLIGKPLQSRIAGYDLFTSLLEKADQKKKRVFFYGAAKHVIAQTIERIERDYPGIEIAGYSDGYVKNQREVADKIAATNPDMVFVALGYPNQEFFIHKYRHLFPQAVSVGLGGSFDVFSGNVKRAPSFFIRFHLEWMYRLITNPARWRRMLSIPKYVTAVLKHERTSAKPQYTGQVKDQSRHL

SEQ ID NO: 25 - protein, 130 aa, Bacillus subtilis
  >ABP10672
MKKVITYGTFDLFHYGHMKLLERARCLGDYLIVGLSTDDFNLQKQKKSHHSYEHRKLILETIDFVNLVIPEKSWEQKITDIKKYGVDTFVIGDDWKGKFDYLNEYCKVIYLPRTEGISSTKIKKEISDLS

SEQ ID NO: 26 - protein, 275 aa, Bacillus subtilis
  >ABP10673
MNALVRIVKEQVTSFPLILRLASYETKSQYQMNYLGVLWQFLNPLIQMLAYWFVFGMGIRNSKPVLTGAGEVPFIVWMLAGLIPWFFISPTILDGSNSVFKRINMVAKMNFPISSLPSVVIASNLFSYFVMMGIYVIVLFASGVYPSMHWIQYIYYLICMIAFMFSFSLFNSTISVLVRDYQFLLQAVTRLLFFLLPIFWNISEQLGKNHPNLLPVLKLNPIFYLIEGFRNSFLDGKWFFQDMKYTLYFWLFTFLLLLVGSILHMKFRDKFVDFL

SEQ ID NO: 27 - protein, 527 aa, Bacillus subtilis
  >ABP10674
MKLKVSFRNVSKQYHLYKKQSDKIKGLFFPAKDNGFFAVRNVSFDVYEGETIGFVGINGSGKSTMSNLLAKIIPPTSGEIEMNGQPSLIAIAAGLNNQLTGRDNVRLKCLMMGLTNKEIDDMYDSIVEFAEIGDFINQPVKNYSSGMKSRLGFAISVHIDPDILIIDEALSVGDQTFYQKCVDRINEFKKQGKTIFFVSHSIGQIEKMCDRVAWMHYGELRMFDETKTVVKEYKAFIDWFNKLSKKEKETYKKEQTEERKKEDPEAFARFRQKKKKPKSLANAVQIAILSILTVFMAGTMFFNAPLRTIASFGAIPQNEVKNHHGNAKGKSEERLTAVNKQGFIANEKAAAYKDQGLKQKADVTLPFGTEVTVAAKGKQAAKIKFDGHSYYVKKSAVAANMKHAELHAAAFTSYVSQNAASSYEYFLKFLGDSRTSIQSKLNGYTEGDTADGRKTLDFDYEKISYVLENDKATELIFHNISPITPASLSLSDSDVLYDSSKKRFLVNTADQVFAVDNEEHTLTLMLK

SEQ ID NO: 28 - protein, 294 aa, Bacillus subtilis
  >ABP10675
MKLKKVRKAIIPAAGLGTRFLPATKAMPKEMLPIVDKPTIQYIIEEAVEAGIEDIIIVTGKSKRAIEDHFDYSPELERNLEEKGKTELLEKVKKASNLADIHYIRQKEPKGLGHAVWCARNFIGDEPFAVLLGDDIVQAETPGLRQLMDEYEKTLSSIIGVQQVPEEETHRYGIIDPLTSEGRRYQVKNFVEKPPKGTAPSNLAILGRYVFTPEIFMYLEEQQVGAGGEIQLTDAIQKLNEIQRVFAYDFEGKRYDVGEKLGFITTTLEFAMQDKELRDQLVPFMEGLLNKEEI

SEQ ID NO: 29 - protein, 509 aa, Bacillus subtilis
  >ABP10676
MKTVFMVVYTIDVNKGGMTTAMLNRSKMLVHNGYKSDLVTFDYNPYYENITSELRQIGKLDPDVNILNVNDYYRDLNTEGNVDPSYYEDEAKTEQEGYFIQDSEYDTKQYIRYFKQGSYVKYKKWTEDGYLSHIDFFNENRQRIKREEFHKNKYKHREISFDPSNNKMNYEKYYTPDGFCYLIRWYNSETEKQQQVFLFNRNSNKVLMFKNNAEFHTYWLNEIAAAENEKPIFICDGPGSSGKVRGMKKELAHRIYMVHINHFETPYTYGSKVKQDHIDFLSNIDKLDALVVLTNDQKKDIEKQFGEHGNIFIIPNSMPYTDLPDIKKDNKKVSMFVRYHKQKAIDEAIKAFVRVIKKVPDARLEIFGHGAEKSRLEQLIIELNLQQNVFIKGYAKNVREEMGSSLITLLTSNYEAFGLSITESFMNGTPVISYDCNYGPRDVISDGIDGYIVPQKDQKALANQIIKLLNNPDLAKEMGLKGREKVLTEYTNEVVLNKWLQLFNVLEKK

SEQ ID NO: 30 - protein, 79 aa, Bacillus subtilis
  >ABP10677
MYDFLNVPQPDYSWIEHPIEEAGLTYIKVPEKPVYRYYGKYVKYQRFSSSVNWLYQVILMTAQAKVQKRRVRKTRTQRI

SEQ ID NO: 31 - protein, 61 aa, Bacillus subtilis
  >ABP10678
MFLTYTNGEGYEHYQYLINELSLIIFEGIFGKISIILSGGAWHFIQNNKASALSFVNHFLS

SEQ ID NO: 32 - protein, 106 aa, Bacillus subtilis
  >ABP10825
MAWFLLVIAGIEEIIAAIAMKYIDGTRKKWPIIVMTVGFGLSFYCLSQAMIVLPAGVAYAVWTGIGSIGVSAVGFIWFKERFQLSQVISLCLILAGVIGLRLTSSS

SEQ ID NO: 33 - protein, 111 aa, Bacillus subtilis
  >ABP10826
MNWVLVFIAGLLEVVWASSLKHADSLLDWIIIFILIAVSFILLIRSYQKIPMAAAYTVFVGIGTVGTYLTGIVLGESFSAAQMFFLALLLAGILGMKLFTKESKSQPGGEQ

SEQ ID NO: 34 - protein, 194 aa, Bacillus subtilis
  >ABP10827
MPKQTSGKYEKILQAAIEVISEKGLDKASISDIVKKAGTAQGTFYLYFSSKNALIPAIAENLLTHTLDQIKGRLHGDEDFWTVLDILIDETFLITERHKDIIVLCYSGLAIDHSMEKWETIYQPYYSWLEKIINKAIANLEVTEEINSKWTARTIINLVENTAERFYIGFEQDENVEVYKKEIFSFLKRSLGTA

SEQ ID NO: 35 - protein, 520 aa, Bacillus subtilis
  >ABP10828
MSKQGNFQKSMSLFDLILIGMGAIFGSAWLFAVSNVASKAGPSGAFSWILGGAIILLIGLVYAELGAALPRTGGIIRYPVYSHGHLVGYLISFVTIVAYTSLISIEVTAVRQYVAYWFPGLTIKGSDSPTISGWILQFALLCLFFLLNYWSVKTFAKANFIISIFKYIVPITIIIVLIFHFQPENLSVQGFAPFGFTGIQAAISTGGVMFAYLGLHPIVSVAGEVQNPKRNIPIALIICIIVSTIIYTVLQVTFIGAIPTETLKHGWPAIGREFSLPFKDIAVMLGLGWLATLVILDAILSPGGNGNIFMNTTSRLVYAWARNGTLFGIFSKVNKDTGTPRASLWLSFALSIFWTLPFPSWNALVNVCSVALILSYAIAPISSAALRVNAKDLNRPFYLKGMSIIGPLSFIFTAFIVYWSGWKTVSWLLGSQLVMFLIYLCFSKYTPKEDVSLAQQLKSAWWLIGFYIMMLIFSYIGSFGHGLGIISNPVDLILVAIGSLAIYYWAKYTGLPKAAIDYDK

SEQ ID NO: 36 - protein, 516 aa, Bacillus subtilis
  >ABP10829
MNYIKAGKWLTVFLTFLGILLFIDLFPKEEHDQKTKSKQKPDYRAAYHFTTPDKWKNDPQKPIYFDGKYHYFYLYNRDYPKGNGTEWRHAVSEDLVHWTDEGVAIPKYTNPDGDIWTGSVVVDKENTAGFGKNALVAIVTQPSAKDKKQEQYLWYSTDKGKSFKFYSGNPVMPNPGTDDFRDPKVIWDDQDNKWVMVMAEGSKIGFYESDNLKDWHYTSGFFPEQAGMVECPDLYMMRASDGANKWVLGASANGKPWGKPNTYAYWTGSFDGKEFKADQTEAQWLDYGFDWYGGVTFEDSKSTDPLEKRYALAWMNNWDYANNTPTMKNGFNGTDSVIRELRLKEQDGTYSLVSQPIEALEQLTVSTEEIEDQDVNGSKTLSITGDTYQLDTDLSWSELKNAGVRLRESEDQKRHIDVGIFAEGGYSYVNRAATNQPDKSNTYVESKAPYDVSKRKVHLKILVDKTTIEVFVGDGKTIFSNEVFPKPEDKGITLFSDGGTASFKNITVKHFDSIHK

SEQ ID NO: 37 - protein, 473 aa, Bacillus subtilis
  >ABP10830
MNIKKFAKQATVLTFTTALLAGGATQAFAKETNQKPYKETYGISHITRHDMLQIPEQQKNEKYQVPEFDSSTIKNISSAKGLDVWDSWPLQNADGTVANYHGYHIVFALAGDPKNADDTSIYMFYQKVGETSIDSWKNAGRVFKDSDKFDANDSILKDQTQEWSGSATYTSDGKIRLFYTDFSGKHYGKQTLTTAQVNVSASDSSLNINGVEDYKSIFDGDGKTYQNVQQFIDEGNYSSGDNHTLRDPHYVEDKGHKYLVFEANTGTEDGYQGEESLFNKAYYGKSTSFFRQESQKLLQSDKKRTAELANGALGMIELNDDYTLKKVMKPLIASNTVTDEIERANVFKMNGKWYLFTDSRGSKMTIDGITSNDIYMLGYVSNSLTGPYKPLNKTGLVLKMDLDPNDVTFTYSHFAVPQAKGNNVVITSYMTNRGFYADKQSTFAPSFLLNIKGKKTSVVKDSILEQGQLTVNK

SEQ ID NO: 38 - protein, 451 aa, Bacillus subtilis
  >ABP10831
MKQNKRKNLQTLFETLGEKHQFNGTVLAAEGGDILYHHSFGYAEMTEKRPLKTNSLFELASLSKPFTALGIILLEEKGILGYEDKVDRWLPGFPYQGVTIRHLLNHTSGLPDYMGWFFANWDPHKIAVNQDIVDMLMNEGLSGYFEPNEGWMYSNTGYVLLAVIIEKASGMSYADFMKTSIFLPAGMNETRVYNRRLSPERIDHYAYGYVYDVHSETYVLPDELEETNYVVYLDGIQGDGTVNSVTSDLFRFDQALYQDDFISKASKESAFSPVRLNNGETIDYGFGWVLQNSPEKGRIVSHSGGWPGYSTLMIRYIDHRKTLIYLSNKEEDTEYEQAILKAAEHILFGQPYEVPERPADKKKKAIDTAIYSRYVGSYLLQDGTAAQVTAENERLYLEIAGQLRLELFPSSETRFFLRALSVEVEFTLGVDAAKSFILYEDGSEEEAVRTK

SEQ ID NO: 39 - protein, 227 aa, Bacillus subtilis
  >ABP10832
MIGILAGMGPKSTSPFIDKVIDYCQKLYGASNDIDYPHMMIYSCPTPFYADRPIDHDEMKKAIIDGAVKLEKTGVDFIALPCNTAHVYYEEIQQALSVPMLHIVEETIKEIPHLAKKAVVLGTEPTIQSAIYQKVLKGNGQEVIHKDHWQQAVNQLIAAIKQPNHMQHTQALWQTLYEEISQHADIIISACTDLNAVLDHIQSEIPIIDSSACLAKSTVSTYLAYQS

SEQ ID NO: 40 - protein, 151 aa, Bacillus subtilis
  >ABP10833
MKKPVLKPFASLEIKVDPPITIGETSLGLRRFIPIRSGTITGEVKGRILPGGADSQMIRANGRTDLSARYVIETADHELIYIENNGIRQVSEPFRKQAAAGEIIEPEHVYFRTVPTFETGSEVYQWLHDRLFIGSAERTPDYVLLDIYEVQ

SEQ ID NO: 41 - protein, 161 aa, Bacillus subtilis [sequence omitted]

SEQ ID NO: 42 - protein, 63 aa, Bacillus subtilis
  >ABP10835
MGKTGYIGAAIVVAACIIILSAVVCLRDTVYYQPMRWTGIILFFAGIVMVPAYSAKRKPGKEK

SEQ ID NO: 43 - protein, 489 aa, Bacillus subtilis
  >ABP10836
MTHQIVTTQYGKVKGTTENGVHKWKGIPYAKPPLGQWRFKAPEPPEVWEDVLDATAYGPICPQPSDLLSLSYTELPRQSEDCLYVNVFAPDTPSQNLPVMVWIHGGAFYLGAGSEPLYDGSKLAAQGEVIVVTLNYRLGPFGFLHLSSFDEAYSDNLGLLDQAAALKWVRENISAFGGDPDNVTVFGESAGGMSIAALLAMPAAKGLFQKAIMESGASRTMTKEQAASTSAAFLQVLGINEGQLDKLHTVSAEDLLKAADQLRIAEKENIFQLFFQPALDPKTLPEEPEKAIAEGAASGIPLLIGTTRDEGYLFFTPDSDVHSQETLDAALEYLLGKPLAEKVADLYPRSLESQIHMMTDLLFWRPAVAYASAQSHYAPVWMYRFDWHPKKPPYNKAFHALELPFVFGNLDGLERMAKAEITDEVKQLSHTIQSAWITFAKTGNPSTEAVNWPAYHEETRETLILDSEITIENDPESEKRQKLFPSKGE

SEQ ID NO: 44 - protein, 152 aa, Bacillus subtilis
  >ABP10837
MIGRIIRLYRKRKGYSINQLAVESGVSKSYLSKIERGVHTNPSVQFLKKVSATLEVELTELFDAETMMYEKISGGEEEWRVHLVQAVQAGMEKEELFTFTNRLKKEQPETASYRNRKLTESNIEEWKALMAEAREIGLSVHEVKSFLKTMGR

SEQ ID NO: 45 - protein, 234 aa, Bacillus subtilis
  >ABP10838
MNENMSFKELYAIVRHRFVLILLITIGVTLMMGFVQFKVISPTYQASTQVLVHESDGEENSNLSDIQRNLQYSSTFQSIMKSTALMEEVKAELHLSESASSLKGKVITSSENESEIINVAVQDHDPAKAAEIANTLVNKFEKEVDERMNVQGVHILSEAKASESPMIKPARLRNMVMAFGAAVMGGITLAFFLHFLDDTCKSARQLSERTGLPCLGSVPDVHKGRNRGIKHFGE

SEQ ID NO: 46 - protein, 227 aa, Bacillus subtilis
  >ABP10839
MIFRKKKARRGLAQISVLHNKSVVAEQYRTIRTNIEFSSVQTNLRSILVTSSVPGEGKSFSAANLAAVFAQQQEKKVLLVDADLRKPTINQTFQVDNVTGLTNVLVGNASLSETVQKTPIDNLYVLTSGPTPPNPAELLSSKAMGDLISEIYEQFSLVIFDSPPLLAVADAQILANQTDGSVLVVLSGKTKTDTVLKAKDALEQSNAKLLGALLNKKKMKKSEHYSY

SEQ ID NO: 47 - protein, 598 aa, Bacillus subtilis
  >ABP10840
MIIALDTYLVLNSVIAGYQFLKDSYQFYDSGALLLTAVSLLLSYHVCAFLFNQYKQVWTYTGLGELIVLLKGITLSAAVTGIIQYAVYHTMFFRLLTACWVLQLLSIGGTRILSRVLNESIRKKRCASSRALIIGAGSGGTLMVRQLLSKDEPDIIPVAFIDDDQTKHKLEIMGLPVIGGKESIMPAVQKLKINFIIIAIPSLRTHELQVLYKECVRTGVSIKIMPHFDEMLLGTRTAGQIRDVKAEDLLGRKPVTLDTSEISNRIKGKTVLVTGAGGSIGSEICRQISAFQPKEIILLGHGENSIHSIYTELNGRFGKHIVFHTEIADVQDRDKMFTLMKKYEPHVVYHAAAHKHVPLMEHNPEEAVKNNIIGTKNVAEAADMSGTETFVLISSDKAVNPANVMGATKRFAEMIIMNLGKVSRTKFVAVRFGNVLGSRGSVIPIFKKQIEKGGPVTVTHPAMTRYFMTIPEASRLVIQAGALAKGRQIFVLDMGEPVKIVDLAKNLIHLSGYTTEQVPIEFTGIRPGEKMYEELLNKNEVHAEQIFPKIHIGKAVDGDWPVLMRFIEDFHELSEADLRARLFAAINTSDKMTAASVH

SEQ ID NO: 48 - protein, 381 aa, Bacillus subtilis
  >ABP10841
MTKKILFCATVDYHFKAFHLPYFKWFKQRGWEVHVAANGQTKLPYVDEKFSIPIRRSPFDPQNLAVYRQLKKVIDTYEYDIVHCHTPVGGVLARLAARQARRHGTKVLYTAHGFHFCKGAPMKNWLLYYPVEKWLSAYTDCLITINEEDYKRAKGLQRPGGRTQKIHGIGVNTERFRPVSPIEQQRLREKHGFREDDFILVYPAELNLNKNQKQLIEAAALLKEKIPSLRLVFAGEGAMEQTYQMLAEKLGASANVCFYGFCSDIHELIQLADVSVASSIREGLGMNVLEGMAAEKPAIATDNRGHREIIRDGENGFLIKIGDSAAFARRIEQLYHKPEICRKLGQEGRKTALRFSEARTVEEMADIYSAYMDMDTKEKSV

SEQ ID NO: 49 - protein, 278 aa, Bacillus subtilis
  >ABP10842
MNSGPKVSVIMGIYNCERTLAESIESILSQSYKNWELILCDDASTDGTLRIAKQYAAHYSDRIKLIQNKTNKRLAASLNHCLSHATGDYIARQDGDDLSFPRRLEKQVAFLEKHRHYQVVGTGMLVFDEFGVRGTRILPSVPEPGIMAKGTPFCHGTIMMRASAYRTLKGYRSVRRTRRMEDIDLWLRFFEEGFRGYNLQEALYKVREDSDAFKRRSFTYSIDNAILVYQACRRLKLPLSDYIYIAKPLIRAFMPAAVMNRYHKKRVMNQKEGLVKHE

SEQ ID NO: 50 - protein, 384 aa, Bacillus subtilis
  >ABP10843
MNSSQKRVLHVLSGMNRGGAETMVMNLYRKMDKSKVQFDFLTYRNDPCAYDEEILSLGGRLFYVPSIGQSNPLTFVRNVRNAIKENGPFSAVHAHTDFQTGFIALAARLAGVPVRVCHSHNTSWKTGFNWKDRLQLLVFRRLILANATALCACGEDAGRFLFGQSNMERERVHLLPNGIDLELFAPNGQAADEEKAARGIAADRLIIGHVARFHEVKNHAFLLKLAAHLKERGIRFQLVLAGDGPLRGEIEEEARQQNLLSDVLFLGTEERIHELMRTFDVFVMPSLYEGLPVVLVEAQASGLPCIISDSITEKVDAGLGLVTRLSLSEPISVWAETIARAAAAGRPKREFIKETLAQLGYDAQQNVGALLNVYNISTEKDHNR

SEQ ID NO: 51 - protein, 367 aa, Bacillus subtilis
  >ABP10844
MIVYAVNMGIVFIWSWFAKMCGGRDDSLATGYRPNKLLIWIPLASLVLVSGLRYRVGTDFQTYTLLYELAGDYQNVWQIFGFGTAKTATDPGFTALLWLMNFITEDPQIMYFTVAVVTYSFIMKTLADYGRPFELSVFLFLGTFHYYASFNGIRQYMVAAVLFWAIRYIISGNWKRYFLIVLVSSLFHSSALIMIPVYFIVRRKAWSPAIFGLSALFLGMTFLYQKFISVFVVVLENSSYSHYEKWLMTNTNGMNVIKIAVLVLPLFLAFCYKERLRSLWPQIDIVVNLCLLGFLFGLLATKDVIFARFNIYFGLYQMILVPYFVRIFDEKSNALIYIAIVVCYFLYSYLLMPVDSSVLPYRTIFSR

SEQ ID NO: 52 - protein, 344 aa, Bacillus subtilis
  >ABP10845
METPAVSLLVAVYNTETYIRTCLESLRNQTMDNIEIIIVNDGSADASPDIAEEYAKMDNRFKVIHQENQGLGAVRNKGIEAARGEFIAFIDSDDWIEPDYCEQMLRAAGDETDLVICNYAAEFEDTGKTMDSDIAQTYQDQPKEHYIKALFEGKVRGFSWNKLYRRSMIDAHRLSFPLRGELEHVEDQFFSFRAHFFARSVSYVKTPLYHYRIHLSSIVQRYQKKLFESGLALYEANAAFLQENNKLEEYRKELDTFIVLHSSICMLNEWKTSGSRRLFEKLRNVGVICADPVFQESLSKTGTAPFDAKRSCLLLMAKYRMIPFVAMASAVYQRVIEYKMRNRG

SEQ ID NO: 53 - protein, 358 aa, Bacillus subtilis
  >ABP10846
MSLQSLKINFAEWLLLKVKYPSQYWLGAADQPIKAAAHQKKIILTLLPSHDNLGDHAIAYASKAFLEQEYPDFDIVEVDMKDIYKSAKSLIRSRHPEDMVFIIGGGNMGDLYRYEEWTRRFIIKTFHDYRVVQLPATAHFSDTKKGRKELKRAQKIYNAHPGLLLMARDETTYQFMKQHFHEKTILKQPDMVLYLDRSKPPAEREGVYMCLREDQESVLQEDQRNRVKAALFEEFGEIKSFTTTIGRRVSRDTREQELEALWSKLQSAEAVVTDRLHGMIFCALTGTPCVVIRSFDHKVMEGYQWLKDIPFMKLIEHPEPERVTAAVNELLTKETPRAGFPRDVYFKGLRDKISGEAQ

SEQ ID NO: 54 - protein, 344 aa, Bacillus subtilis
  >ABP10847
MTPLVSIIVPMYNVEPFIEECIDSLLCQTLSDIEIILVNDGTPDRSGEIAEDYAKRDARIRVIHQANGGLSSARNTGIKGARGTYIGFVDGDDYVSSAMFQRLTEEAEQNQLDIVGCGFYKQSSDRRTYVPPQLEANRVLTKPEMTEQLKHAHETRFIWYVWRYLYRRELFERANLLFDEDIRFAEDSPFNLSAFCEAERVKMLDEGLYIYRENPNSLTEIPYKPAMDEHLQKQYQAKIAFYNHYGLAGACKEDLNVYICRHQLPMLLANACASQNSPKDIKKKIRQILSYDMVRQAVRHTPIQHEKLLRGERLVLALCKWRLTFLIKLFFEQRGTMKGSAKQA

SEQ ID NO: 55 - protein, 482 aa, Bacillus subtilis
  >ABP10848
MTPFIVKTLGVEAFGFVHLTQNVINYFSIITVALSSVVVRFFSVAAHRGEREKANAYISNYLAASVLISLLLLLPLAGSAFFIDRVMNVPQALLADVRLSILIGSVLFILTFLMAGFGAAPFYANRLYITSSIQAVQMLIRVLSVLLLFACFAPKIWQIQLAALAGAVMASVLSFYFFKKLIPWFSFRMKDLSFRTSKELFQAGAWSSVNQIGVLLFLQIDLLTANLMLGASASGKYAAIIQFPLLLRSLAGTVASLFAPIMTSYYSKGDMDGLMNYANKAVRLNGVLLALPAALLGGLAGPFLTIWLGPSFSSIAPLLFIHAGYLVVSLAFMPLFYIWTAFNQQKTPAIVTLLLGAVNVVLAVTLSGPAHLGLYGITLAGAISLILKNAIFTPLYVSRITGYKKHVFFKGIIGPLSAAVFAWTVCKAIQFIVKIDSWPSLIAAGVTVSFFYAVFAFMLVCTKEERQLVLKRFRKTKGAVNL

SEQ ID NO: 56 - protein, 202 aa, Bacillus subtilis
  >ABP10849
MILKRLFDLTAAIFLLCCTSVIILFTIAVVRLKIGSPVFFKQVRPGLHGKPFTLYKFRTMTDERDGEGNLLPDEVRLTKTGRLIRKLSIDELPQLLNVLKGDLSLVGPRPLLMDYLPLYTEKQARRHEVKPGITGWAQINGRNAISWEKKFELDVWYVDNRSFILDLKILCLTVRKVLVSEGIQQTNHVTAERFTGSGDVSS

SEQ ID NO: 57 - protein, 216 aa, Bacillus subtilis
  >ABP10850
MKNVAIVGDGGHGKVIRELINARSDTRLAAVLDDKFKTFEGGKEWYTGPPEAVTELRRLIPDVLFLIAVGNNSVRKQLAERLGLRKDDFITLIHPSAIVSRSAVIGEGTVIMAGAIIQADARIGAHCIINTGAVAEHDNQISDYVHLSPRVTLSGAVSVQEGAHVGTGASAIPQITIGAWSIVGAGSAVIRPIPDRVTAAGAPARIISSIQTSNKG

SEQ ID NO: 58 - protein, 388 aa, Bacillus subtilis
  >ABP10851
MHKKIYLSPPHMSGREQHYISEAFRSNWIAPLGPLVNSFEEQLAERVGVKAAAAVSSGTAAIHLALRLLEVKEGDSVFCQSFTFVATANPILYEKAVPVFIDSEPDTWNMSPTALERALEEAKRNGTLPKAVIAVNLYGQSAKMDEIVSLCDAYGVPVIEDAAESLGTVYKGKQSGTFGRFGIFSFNGNKIITTSGGGMLVSNDEAAIEKARFLASQAREPAVHYQHSQIGHNYRLSNILAGVGIAQLEVLDERVEKRRTIFTRYKNVLGHIAGVRFMPEYAAGVSNRWLTTLTLDNGLSPYDVVQCLAEENIEARPLWKPLHTQQLFDPALFYSHEDTGSVCEDLFKRGICLPSGSNMTEDEQDRVIEVLLHLFQTAEVKKWTASIR

SEQ ID NO: 59 - protein, 322 aa, Bacillus subtilis
  >ABP10852
MDSKHSMISLKQKLSGLLDVIPKQSEIIYADYPLYGNVGDLFIMKGTEAFFKEHGIRVRKRWNPDNFPVGRKLDPNLIIVCQGGGNFGDLYPYYQGFREKIVQTYPNHKIVILPQSIYFQNKDNLKRTAEIFSKHANLHIMTREKASYATAQAYFSKNHIQLLPDMAHQLFPVIPTQQPSNQKLRFIRTDHEANQALQEHTETESYDWRTVLSASDRRTIAFLQTLNVLNKKAGNPLPIAYIWGKYSDYIVQKAIRFFSRYESVETSRLHGHILSALLQKENTVIDNSYGKNANYFHTWMEGVPGTRLIQHASKKENLPAHM

SEQ ID NO: 60 - protein, 72 aa, Bacillus subtilis
  >ABP10853
MSELFSVPYFIENLKQHIEMNQSEDKIHAMNSYYRSVVSTLVQDQLTKNAVVLKRIQHLDEAYNKVKRGESK

SEQ ID NO: 61 - protein, 39 aa, Bacillus subtilis
  >ABP10854
MLTPLSSLYMIEITPYTFMKKELPKKCLNFFPSLILLRI

SEQ ID NO: 62 - protein, 437 aa, Bacillus subtilis
  >ABP10855
MMDMKLQQVQVLKPQLTQELRQAITLLGYHSAELAEYIDELSLENPLIERKETDTPPLSYHKTNKNRMNAQEAGLQLSNPQKTLQDALKQQSLDMNLTNTEKKIFNYLIHSLDSNGYLEEDVEEAARRLSVSAKETEAVLAKLQSLEPAGIGARSLQECILLQLQRLPNRNEQAEMLVSAHFDAFAQKKWKALSVETGIPLHTIQDISDDIAALHPRPGLLFARPEQDVYIEPDIFITVKNGHIAAELNTRSFPEIDLHPQYRTLLSSGSCQDTVSYLSAKYQEWRWLSRALRQRKQTITRIINELITRQKDFFLKGRSAMKPLTLREVADCLSLHESTVSRAIKGKTIQTPYGLFEMKLFFSAKAEASGEGDASNYAVKMHLEDLINQEDKTKPLSDQKLVDLLYEQHGIQISRRTVAKYRDQMKIPSSAARKRYK

SEQ ID NO: 63 - protein, 563 aa, Bacillus subtilis
  >ABP10856
MQWTQAYTPIGGNLLLSALAALVPIIFFFWALAIKRMKGYTAGLATLGIALIIAVLVYRMPAEKALMSATQGAVYGLLPIGWIIVTSVFLYKITVKTGQFDIIRSSVLSITDDRRLQALLIAFSFGAFLEGAAGFGAPVAISAALLVGLGFNPLYAAGICLIANTAPVAFGAIGIPITAVEGPTGIPAMEISQMVGRQLPFLSVFIPLYLIIIMSGFRKALEVWPAILVSGVSFAVVQYLSSNFLGPELPDVLSALVSMAALAVFLKWWKPKTTFRFAGEQESAASIETARTNPAAPAYSGGQIFKAWSPFLLLTAMISVWGIPSVKSALTGHYEGSAVFLKWLNAVGEKLTFAPGVPFLNNQIVNADGTPIEAVYKLEVLGSAGTAILIAAVLSKFITAISWKDWGTVFKETVQELKLPILTIASVVGFAYVTNSSGMSTTLGMTLALTGSMFTFFSPVLGWLGVFITGSDTSANLLFGNLQKVTALSVGMDPVLSVAANSSGGVTGKMISPQSIAVACAAVGLAGKESDLFRFTIKHSLFLLLLVCIITFLQHHVFSWMIP

SEQ ID NO: 64 - protein, 240 aa, Bacillus subtilis
  >ABP10857
MKYKQIKTKKIYEEVADALLDMIKNGELKPGDKLDSVQALAESFQVSRSAVREALSALKAMGLVEMKQGEGTYLKEFELNQISQPLSAALLMKKEDVKQLLEVRKLLEIGVASLAAEKRTEADLERIQDALKEMGSIEADDELGEKADFAFHLALADASQNELLKHLMNHVSSLLLETMRETRKIWLFSKKTSVQRLYEEHERIYNAVAAGNGVQAEAAMLAHLTNVEDVLSGYFEENVQ

SEQ ID NO: 65 - protein, 332 aa, Bacillus subtilis
  >ABP10858
MATIKDIAQEAGFSISTVSRVLNNDESLSVPDETREKIYEAAEKLNYRKKTVRPLVKHIAFLYWLTDKEELEDVYFKTMRLEVEKLAKAFNVDMTTYKIADGIESIPEHTEGFIAVGTFSDEELAFLRNLTENGVFIDSTPDPDHFDSVRPDLAQMTKKTVNILTEKGHKSIGFIGGTYKNPNTNQDEMDIREQTFRSYMREKAMLDERYIFCHRGFSVENGYRLMSAAIDILGDQLPTAFMIAADPIAVGCLQALNEKGIAIPNRVSIVSINNISFAKYVSPPLTTFHIDIHELCKNAVQLLLEQVQDKRRTVKTLYVGAELIVRKSMNEG

SEQ ID NO: 66 - protein, 421 aa, Bacillus subtilis
  >ABP10859
MKMAKKCSVFMLCAAVSLSLAACGPKESSSAKSSSKGSELVVWEDKEKSIGIKDAVAAFEKEHDVKVKVVEKPYAKQIEDLRMDGPAGTGPDVLTMPGDQIGTAVTEGLLKELHVKKDVQSLYTDASIQSQMVDQKLYGLPKAVETTVLFYNKDLISEKELPKTLEEWYDYSKKTANGSKFGFLALFDQIYYAESVMSGYGGYIFGKAKDGSYNPSDIGINNEGAVKGAALIQKFYKDGLFPAGIIGEQGINVLESLFTEGKAAAIISGPWNVEAFSKAGINYGITKLPKLENGKNMSSFIGVKSYNVSAFSKNEELAQELAVFLANEKNSKTRYEETKEVPAVKSLANDPAIMKSGAARAVTEQSRFSEPTPNIPEMNEIWTPADSALQTVATGKADPKQALDQAAETAKGQIKAKHSGK

SEQ ID NO: 67 - protein, 418 aa, Bacillus subtilis
  >ABP10860
MQHRQVALLLSIIPGLGQFYNKQWIKGIVFLFLGASFFAVFGDLLNMGFWGIFTLGTEVPRDNSVFLLAEGIIAVIVTCFGLAVYYVNLRDAFQSGKQRDENKPLSSLKEQYQHIISEGYPYVVSGPSLFILIFAVIFPILFSFALAFTNYDLYHSPPAKLIDWVGFQTFANIFTVDIWRSTFFDVLAWTVVWTLAASTLQVSLGIFLAIIVNQKDLRFKRFFRTILILPWAVPGFVTILIFAGLFNDSFGAMNHDILAFFGIDPLPWMTDANWSRLALILMQGWLGFPYIFLVSTGVLQSIPDDLYEAATIDGASVFSKLRYITLPMVFIAMAPIIITQFTFNFNNFNIIYLFNGGGPAVTGSTAGGTDILVSWIYKLTMQSSQYSLAAALTILLSVFVISIALWQFRQTKSFKEEA

SEQ ID NO: 68 - protein, 52 aa, Bacillus subtilis
  >ABP10886
MRKDKLVSTVFKNNAIEIYTIIILKNPDTLVRIKEIQLFHTKKSLAASAAKL

SEQ ID NO: 69 - protein, 1015 aa, Bacillus subtilis
  >ABP10887
MFPEVNDKDELQKIFLNVSGKTIHSLIRDDTNIEQNTNIIDIDRVLDHKKSDFLVRNSEEFLEHNPFFHFFSPFLSCKIEEFIVKVRIEDAVDNEDEFVKKVIKHILDLMFEKAFRVLVLEVNIARLEGKLEGTTPEERLNHFLAVSLNDESFLKSVYKEYEVLTSLLCVTIDDYFTYVMEIIKNTKREISSLNSKFNSDNDLGAITNITTGLGDTHQKGKSVSTIYFKSGKKIIYKPRDLTLEQGFQEVLYWLDGKNIPGILNFKRVQIHTVNDSGWMEHIDYKSCFNKNEANDFYTRSGNLLCLLYLLNAVDFHHENLIAHGSFPVLVDLESLFHARLKVDQIDKKSAFVTATELVDNSVQSISLLPTKISKRVGDKDISLDIGGLGAYKEQLSPHKSLVIENAGTDTIKILRKNTFIKPQLNNPSIKTGSYLYSENYTGQIKDGFESLYSWVMLNKDEFWDKISQTFKETNSRFIFRPTYLYTQLLRISSHPDFMRDTYRRKIILHRIGIDYIQEYKDILNSEYKDLLTGDVPFFRSSIEHEHLIDSRGGKIHNILEEPPIKTVKQKIFNLSKEDLKRQIDFIEMSYISNEKRLKEVTDIKFSKAANLNKIKSENWIDEATQIGEFIVENSVCGINKKQKDRMWIGPSLEGIEEDIWNANVLGFDIYNGNSGIALFLGYLGEILNRQDFKQAAIETMRPIQKFISEIKEDHPYLIGAFQGISGYFYTLNKLSNLFEDSELRKTTLENISVLSKLGKFDKVYDLIGGSLGSLAVMLSIIPNITEENNKKEILKISHIHCDHILSVAKNFEEQISWPGKFSAAYSGFSHGNSGFIAYLYKFFKLTNDEQLLEVIQRALRFERRLYSEDHNNWYTTENKDKLANGWCHGAPGILLSKLILKDNGFEDEYIEKEISTAIDSSIHNGIGNNPTYCHGDLGVLSILNYASDLTNNINLKNRCLRTYQDLFENVLAMKWRKRDLVCTRSYSLMIGLSGIGYSMIKNYAPEIVPNFLWLE

SEQ ID NO: 70 - protein, 66 aa, Bacillus subtilis
  >ABP10888
MKKDMVKNASGFIEEDELISLANGENATGGGTPVTAIITALTGTTFTVTLSAASCPTSACTNLCNK

SEQ ID NO: 71 - protein, 982 aa, Bacillus subtilis
  >ABP10889
MDISYENNNFIRDAVINFSSPTNEVEKLRIKNKDYFGNFYTFFLDFYQQRLFNTLENASKENNLKLNKQKIISSALEAFSQELIQLCIRTLIVDINDRKEKGLLEGKDSKLRYKNYNNLIFKSEYVAEILNKYPVLTYLISSRISNKILYLKEVLENLRKNRQDIYRELRIEFDEVSNIYFSSGDTHNGGKNVLIIETNQGKIVYKPHSLSPDILFNSIVDYVNNSDKILKKIYKIRTLNYKDYGYQEFIDYKECETSEKLNFYFYRVGVSLSIFHIIGCDDLHHENLIAHGEYPVVIDLETLIKNNSIYKPRNNNLIDNFHEDINYSVLGTMLLPLNLQTSIFDFDLGGISNDENQTSEIWKSYIIDFEGTDEIQLTKKSVIMNSTQNRATYNGKAADPKNYIEEILKGFTDCYNFVLENISGFHDLVKKVGSSNLEVRQVLRATSIYARFLEASTHPNYLSSFEERKKLFKKINIAEGVTDKFSKKNLYELESLMCNDVPYFSTMYNSLDLICNKSTSIVNFFRESLLDVVLNKTKSISKASLKKQQYYIRMSLTTTIKDSWKKTNKHNKKYRPKLFGNNNKNYLECATEIGDLFLETAIWNNDRSKCTWVAPIISENNKVKLGPLNFDLYEGGGVILFLALLGKENGKKEYFDLALAGMRGIEELFLSDDKMDDRLSLFTGIGSLSYIYYHLYTHTNDYKYYEKFKKYIKKINEMNISGDIALDIVGGVSSLIVFLLNLYKETKLDILNSVCCKLGNTLYQCLENDKHNYLTGLSHGYSGFTWALCYLGHITKEEKYTTLGKELLKIENKFFDLHTSNWKDLRVGEGNSDPVYWCHGAGGIALSRAFLKDLLKNKENVVDKEIDKEVDRDLSSAICKLLSDGFKKTTDHSLCHGSFGNIDILLKLSEFLNDIDLQEVAFKEAQNAINYIRDKGFIPGLQDHFDLNTFMLGLGGVGYSLLRLHNPVNPSLLAMEVRSYNE

SEQ ID NO: 72 - protein, 715 aa, Bacillus subtilis
  >ABP10890
MIVKKKKRIPIVKQLQQTECGLCCCAMLIRFYNSNETLFELRSFLEAGRDGLTIKQLKNLLVHKGFKADIYKSTIPGLKKINVPFIAYWNNEHFIVVEKTKKNFYYIIDPANGRRKLTEEEFRKGFSSYILYAVPSENFTPNKRKDKNVWFGVLKNITNYKLLFSIIVFLSLISYLLTLYVPILVQKLIDTSIEHNNLNSISNIVWITFLISILYGMFVLFRGLKMISLNIFLSKNLVVDTFAHLLKLPFKFFDLRSPGDLLFRLNSMNGFRELLSTQLISGLIDLGAVVFILAYMFFKSIPLTLITILIFAINTIFMFLTRPAVAQAIDDEVAEQSKSQAIQIESIFSIAAIKISGMENEIFSTWNNSFNDVIKRFKKRSILQNIVNTVTQVFQTIAPLVILILELLLFFDNKFTMGEVIAYHSLSVTFFGLTTSLFGTYTQFILATSYLERVKDITETECEKNFENAVNLKLRGNVKLENVSFSYTKHSPKVLKNISLEIREGQKIAIVGSSGSGKSTLSKLIMGLYDPTEGQICFDSIPLEKLDKKQLYKQMGIVPQDITLFNSSILKNITLNNKNTSIEKVRKVAKAAQIDKEIESMPMKYNTPISEMGMNLSGGQRQRIVLARALLNDPKILILDEATSSLDLVNETLISKYLSEMGCTRVVIAHRLSTIMDSDFIIVLDKGEVVEIGKHEELIALEGVYSNLYRSQMKR

SEQ ID NO: 73 - protein, 56 aa, Bacillus subtilis
  >ABP10891
MKNYKGDGAVFLVIGFCLGLFMGVVFDILPYGLSLGILIGSLIDFYFYARYKNNKK

SEQ ID NO: 74 - protein, 84 aa, Bacillus subtilis
  >ABP10892
MSMSRKETPDDNAFIESFHSSLKSKTLYLNSIERTSTIIVERNVKDYIYYNNIPYSNETKQPITDKLSAIGCLKGVLIPVSKTG

SEQ ID NO: 75 - protein, 427 aa, Bacillus subtilis
  >ABP10981
MIDVIRVSGGYGRKDVLQDISFAVKPGEFLGILGPNGSGKTTLLKMLSGSITPRSGEVLLECRSVGSYKTKELARKVAALPQKTEQAFSFTVEETVQFGRYAYQSGLFRQLTGEDHDIVKRVMKQTDILRFAKKSIHELSGGEQQRVYVAQALAQEPRYLLLDEPTSFLDLSFQKSLLDLIKQETVASKLAVIGVFHDVNIASLYCDRLLLLKDGKAEVLDRPEAALCADRIERVYHTDITALDHPERANPQFTIKAKTIPEKAEPLFLKERIEQYLPRGITFSADRPMRVLSSEEGFAWRRKLVFDSGNNSGWPHDLSTVEQEALFIQHDCKLTACHIVSESNDLCIIGMKDAKGRFIMWVVVSGCLHDGQFVKVISATAKAAAQHRVFCSDVLIAATHSGRLPDQTILLTQIQDQTAACVKALKN

SEQ ID NO: 76 - protein, 300 aa, Bacillus subtilis
  >ABP10982
MKVEGIIPAILTPITKEQDFHPGVAEKLVNHLIDSGVHGIFALGTNGEFHLFSQEEKLQIAETVVKAVNKRVPVFIGAGENSTEATISLSNQMADIGADVLSIITPYFVAPSQKELYQHFRTISENVALPVLLYNIPSRTGVSLEPETVERLAALPNIIGIKDSSGSFDNIKAYLERTKDQSFSVLAGTDSLILDTLKAGGTGAVAATANVLPQTVVSIYESYKQGNIEESEQYQKQLDPLRATFSLGSLPAPLKKATELAGIDVGPPKHPIAELSGEGLQKVKKMLEGYGIETKLVKEQ

SEQ ID NO: 77 - protein, 390 aa, Bacillus subtilis
  >ABP10983
MKTLYHFQTAARIEAGAHSLNFLGDHLDQTSGWNQIRSVFILTQPSIVSLGYADQIKEVLAEKGISSEINTDIQPEPTEQNIEEVFQLFSAGSHDAILGIGGGSVLDAAKILSVLKTNKKPISELVGTNLVEKPGVPLVLIPTTSGTGSEVTPNAIVTFPEKELKIGMVSPYLLPSLVILDPVLTIGLPKAITAATGMDAFTHALESYISNKANPFSDMFALESMRLISSSIQEAYHHGDKLEAREKMLIGAMYGGMALTSAGTAAVHAMAYPLGGKYKMSHGVANSMLLPHVTAFNADHVTDRLSDVAGVIGIEQKGSKASQAERVIQKIEEWTADLNIPQNLKAFGVSKEDVPTLAEAAADVKRLMDNNPKPMSVAEIEAVYLKLLEV

SEQ ID NO: 78 - protein, 467 aa, Bacillus subtilis
  >ABP10984
MDVLSGSVITFILAVIVVYILFTTWLTMRFRSKSSAEFNNAAKTLPAIVVGILLMSEFIGTKSTIGTAESAYTHGLAASWSIVTVSIAFFIFSYFLVGKFYKTGQYTISGIISDKFGRSTKLVVSTIMIVALLLVNLGNYLSGSAAISSILGLPLMTCAIITAIVSTFYFTFGGMKGVAWVTILHSLVKYVGVLITLGVALYLTKGWEPMTQQLPEHFFTWDGSIGWGTIGAWFIGNMGAIFATQFIIQAITSSKSEKEAKRSTLYAALLCLPLAIAIGVIGVAARHLYPDIDAIYAFPVFMQQMNPVLSAIVATSLVASIFVGVSTVALATTTLIMDDFYVPKAKPTPEQRMKVTRYASIIIGFIPLLGVALAPELLTLSFFTRALRTSIAVVAAMGFYLPYFNSNRGATIGLVLSGMATTVWYLLDNPFGIDNMYIAIIVPFVVLVLDRLISSPAKKESNVKEEF

SEQ ID NO: 79 - protein, 392 aa, Bacillus subtilis
  >ABP10985
MKQSEVSLLIDGRIRKNETDEARKDAFLPTDCPQNHAANLLELDNGDLLCVWFGGTQEGIADISIYMSRLAKGSSEWTQIEKLSDDPSRSEQNPVLFQEPSGRLWLMYTAQMSGNQDTAIIRYRTSDDRGHTWSGIDTLFGEAGTFIRQPLVVLDNGDWLLPVFYCITLADVKWTGNRDISAVKISSDKGKTWEEVKVPSSMGCVHMNIEKLHDGTLLALFRSRFADSIYASRSIDNGRTWSEPEPTELPNNNSSIQFTALQDGTLALVYNHMKANETTERRASLYDEIEDEDDTRTGVDTEARPAFWGAPRAPMTLALSHDGGVTWPVKRNIEVGDGYAMTNNSKDKLNREFSYPSIKQGKDGDLHIAFTYYRQAIKYVRVPQMWASADQE

SEQ ID NO: 80 - protein, 594 aa, Bacillus subtilis
  >ABP10986
MKIKVLGIAPYKGLGDLLTELAKEEQDIQFQLEVGDLRSGVAIAEQAVSQGIDIMMSRGGTASLIQKHVRIPVVDIPVSGYDLLRALTLIKDYQGKAAVVGFENITQGVRTISELFGIEVDLYTIKEEMEVWDLLRDIQQQGTQIVLGDVITDKAAKELGMQSMLITSGRESVKEAFHTAKQMYRLFKEASEEQRMFRDMIDQEEKGMLVIDDNSRVRFVNKMVKKWMKEGLLEPIAPAAAVNEWWDELAFAVQSIREGKLSGYFQLETGEVVWHMKGSFLSKGELLIAIEQSSSSRDDRNHPVWSFAAPVHSLHPFSSFTQQSSSMRDTVQQAQAFSQTHKPILLYGEEGTGKSDLALAIHQMSPRRQHTFMTIHCSKVKETSLLKALPAVQNGTIFLRYVEHLPLEVQHDLALQWMKPDQQIRWLASSSADLCEEMKAGRFDPDLYSCLQGLTLYVPSLSERVEDMEDMSRLFIAEFNSVYGTQVVGLAPEVMDAFRNRTFRENVRQFKRVLEELALTVKSGYITLAEAAPQLDRLSNEKKEESLKGYTEGTLEDIERRIIQAVLQEENMNQSKAAKRLNINRTTLWRKLKE

SEQ ID NO: 81 - protein, 446 aa, Bacillus subtilis
  >ABP10987
MTNIRCKKGANISRKILIVADDLTGANDTGVQFVKAGMSAAVLFDRSGANPGDIKEDVMILDTDTRGVSPSEAYKEVSSASHPFARLESHLFLKKIDSTLRGNIGIEIKALMDLGRFDVAVIAPAFPDARRITVDGMHYVNGLPVHETEAAVDPKTPVAESRIADLLFGQTNIQPKTIGTKQLHKPDEQIQQDLRAWKTQGHEWFVCDAETNEDLRRIVQVFMNSGQSVLWVGAAGLAGALAQHVRKRALQTGKRNEPVMIVSGSASNTTNRQLAYVREQRDLLDVRINPLNVLNGCEAWEHKRAIDQVVVHQGKDVLLYTDAKPETVQRIIAFGRKQGLDRQAVGEKLSLFLGAVTSEIVKLTGLKRLVLTGGDTARAICNELGADGIQLLGEIEAGIPLGKLLNADIYAVTKAGAYGQTDSVLRAVEVLRNVEEEDRWQNQSLR

SEQ ID NO: 82 - protein, 335 aa, Bacillus subtilis
  >ABP10988
MAKPIIALTMGDAAGVGPEIIIKAFEQTNLHENGTLFVIGDYSILNRAKTFIGSDVDIVKINEPEEAADVKPGVIPCLDLQLLTDELRVGEVSAEAGNAAFRYLEKAIALANENQIDGICTAPLNKEALHKAGHMYPGHTEILAELTQTKDYAMMLAAPNLKVVHVTTHVGLLDAIHLIDAKRVYTTIQLAHDTLIRAGIPQPKIAVCGINPHAGENGLFGHGEEEEKIVPAVERAQSEGIQAFGPLPADTLFFRAVRGDFDMVVAMYHDQGHGPIKVLGLEAGVNITVGLPIIRTSVDHGTAFDIAGTGKADPASLEEAVRQAIMLSGTRNRHA

SEQ ID NO: 83 - protein, 248 aa, Bacillus subtilis
  >ABP10989
MEFYKKTAIITGASRGIGRAIAETLADKGANVVINGTNEELLKSMCTELNTERKCASYVAGDASLPETASLLIAEAKQQFGQIDILVNNAGINLRKTTVDTSLEEWKRVIDLNLTGIFLMCQAVIPEMTAQGGGKIVNMSSTTSKTPHHNASPAYGASKAGINYLTMHLAKELAAHRIHVNAVCPGPIETDMSKQWSEEYRAAVVERIPLKMIGSPEHVANIVAFLASDKSDFMTGETININGGTYMN

SEQ ID NO: 84 - protein, 51 aa, Bacillus subtilis
  >ABP11306
MSPPNEAPIIPLDCGSLVTFQFSSISGMNWFVCQTHSLMELAFYYLRDRIP

SEQ ID NO: 85 - protein, 272 aa, Bacillus subtilis
  >ABP11307
MKKLIENTENPRTTQSIKKDLEGLGLNKGMTVLVHSSLSSIGWVNGGAIAVIQALMDIVTEEGNIVMPSQSVDLSDPSEWHYPSVPEKWWDTIRESMPAYNAQYTPTTGMGKIVEVFRSYPEVKRSCHPNYSFIAWGKDKNKILNKQSLNFGLGEQSPLGNLYMDNSYVLLLGTDFDSNTCFHLAEYRIPFQKVVIKGAPVLINGKTVWKKYKDLEFREDLFEEIGKSFEIESDMKSGKVGSANCRLFSLKEAVDFAEKWFIEYDCKMNSRG

SEQ ID NO: 86 - protein, 504 aa, Bacillus subtilis
  >ABP11308
MSNYRDYILKGKDVAVFEIDTDPISLDPAKCDDYIGQIISQAMFEPLFIRDIETEQWVCGAAENFEVSSDGLTYIFNLRKDRFWSDGISVVAQDFVFAFQRLFHPKINSPIGQILSFIKNGEEILNGVLPVTELGVEALGPRKLKISLTECLPFLPSILGSPNTSPFPYRTEQVSWTDERLNITNGAYVLKEYKSGQFVRLERNPFYPNSSSNHVKDVLFVINRELDYSLQNYEKGNIDVTCNTYFPFEEIKRFKQRDDFYMFPSGILFFLQFGNRNDLFKKKQARQALYYIVNKSQIAQTLHGGIIPWDHFASIGVSEKLFDDQSNYCYHPEKAVKLWKQEERENQALSILYADFFPNGEICHSIKSEMEKHLGITLTLEGCSFEDFVIRHEQREYDLCLALLSPLYNDPFNYFQYFLSELSEEDEDEFIDILQKALGDEKENHCTYYKKANDYLLEKLPSIPLFNGQSIFLKNPFLKGYKIFKDGSISIQNLSWGTEEKPKL

SEQ ID NO: 87 - protein, 341 aa, Bacillus subtilis
  >ABP11309
MYKLADRIQIVSLHNGRIFLIDDEITELEGSPQHTEKALKLLEKGCMEEELNRIMPLEDTQKLLEFLKEEELLRENWENEYLDTIVEKQLYYLDDFSIDSNQLQSNLKSAKVVILGVGGVGSVLIQHLIGAGIENFILIDNDVVNIHNLNRQFLYTQEDFGKPKVKAAENFMRKVNPSVKVTSYQTTIDSIKSLDFLASHSIDIFINAADYPKHLDKIVDEYCFERKIPWVGSGVGRHQGFWGPLFVPGKTCCLNCFIAEEEKEMKEIEKIIRERSNSIIQASFAPTNTIVSAFLAMDVIHFLAQINQIHSYLTRCQIDFTTLKLNRFTIDEPKLCNCGGE

SEQ ID NO: 88 - protein, 464 aa, Bacillus subtilis
  >ABP11310
MLSKNYSFSLSISHLKSKSDNHQRVQEIFGVTDTQLNNRLIFKNITFLMHDVTYITGFSGSGKSTLVNLIKKDFPDAVIPTPPAKQDIPIIDLLDLELQESMKILGWVGLGEAYLYLTPYSALSEGQKTRFLLAMALSRNPSIIIVDEFLSNLDRITAKVVAYSFQKICRKQEIHLIVASAHNDLIEALAPDILIDLDLNGTHRITNRPIEKPFVPDISGVQVESGTIKDYEELKRFHYFGDEDLFVDNEFETEIFTIRLKEKCIGVSVMKSPYPKDWEEIDYFKDINDRIRCLVRLIIHPSFRTIGLSKLLMRPKFLDVPYIETRSALGLYMPIYLSGGYSRTELPDNKLSPLRQKLWNNLSFMGLSDVHLLRDDIYCENFVQNLSGKQKEALRYLALNVYVEMMVNNYIYFRSISKMIPLLPKEMDELKEMFLDVSDEIPVTVLLQETSLFKMQGFVVQHKQ

SEQ ID NO: 89 - protein, 404 aa, Bacillus subtilis
  >ABP11311
MPLFSTNKNVSFIYLTSCFGNGFFERGIWMLFLIEKGFSLFQIGLLQAFVNGTMFLFEIPGGMLADRYGRKVSLLIGRFMIMSYLLIIMIADSFESLALSFCLLGLGMTFISGSEESLLVDSVKEQTGENNFSRFLGRYMAIITVALSLAMMIGGFLKEISWSLVFAVSFIFQMVAFFGCFFLKETKYKKGSQRESFTLIFKDTFNFLKTNNTSRTLIFGIALFTGIGSIFYMFAQELFNQLGIKVYLISIFFGLESFLAAILADRAYILEKKFSSRGVMMVCVYLCGISFLLIYINFNWLILSFFIISAFYNLFTTISYSVINQDIPSKQRATLLSIISFISSLVMFISIPIFGYLSDKFGTAYLLSFTGVISMVLVALSILSFYKNRKDSVEKHKLLKVQEK

SEQ ID NO: 90 - protein, 269 aa, Bacillus subtilis
  >ABP11312
MEKKLSHHPIDRRVDLTYDEFMKEYGLPGKPVIISNAINNWEAKKLWTLDFFREKYGHIIVPIFESGKRYELYETTLGEYIDYILKEEQEDGIFNLADWEFSRDCPELREHYQVPNYFQSWLEDAPISLLPALRWIYINQKNTGSGLHIDYGHTASWNAVISGKKKWILLNQNESENIYNGAVDAFNPDFKKFPLYTHSQTFYGEQSEGDIMYIPSGWWHQVHNEELTIAVTENFINETNYKNCLWPLVSNIVEYQLEISKTPEKVQKV

SEQ ID NO: 91 - protein, 388 aa, Bacillus subtilis
  >ABP11821
MGGGLYGHRNIEDERLKEWIKTWKAENYIHFFCNYYGVGMNAEFNDSLAKQVELVIQESSSITVSKDRYLFDEVMKYMTPEMFYCYFRYDSSTAYCGNYYEVLIEFADELTKKKLIKGYDYVQTGGITLEKNGEVIGHIGQMSDLFWQTFYDQYIVEDYGAIEHARNNGKDITLQIWNDKVFENTEQFYKFIEQILFECNVNLGFGFKMSRFENESKLKGHTSNTKLCLSNIELEETPLRYFNFANYTKIPRHKYLAYYQVIEFFFTRAVRKARFPQPNELLIVKYIATNSITELEVVTWLDDIKSRGKHYTKPSEKYPALFPLEATEIVESVAKRIYLIRCSLVHSKEAPNDVNFIPNLNDEIIDKEISLIKYVAEKVLYKWSNAPE

SEQ ID NO: 92 - protein, 130 aa, Bacillus subtilis
  >ABP11822
MLESTYLQITDVIGKIIPADWSKIVLYAEILDGSREVYFFFQTPENDEYIYSHDIPEQFQVSKKIYTELLIDLQELFKQLHNEFKENNPEAWTNLTLNLESNGTFSIDYNYDDVLSSELDDLQRRDVWKC

SEQ ID NO: 93 - protein, 162 aa, Bacillus subtilis
  >ABP11823
MENELNALYRSIAETVNEMIPEPWEKFLFYAQVSETGGGTYFFYNSQNEPNHFKYSLEIPFEFDIDENEFDQYEMELFKLSEKMRDVFKDHDQELFYSFTLSLERSGKLTVNFDYTDWFKTDYSFSDQLIIWKFKYLGEEPKDPSLQKLIKKYLEEYPENPI

SEQ ID NO: 94 - protein, 669 aa, Bacillus subtilis
  >ABP11824
MKVFEAKTLLSEATDRAKEYKELRTQMVNLRKALKSVADLSDSEFSGKGASNIKAFYHDHVGVTDQWIDYIDMKIAFFNSIAGAAEDKALSDAYIEESFLEHELANANKKSKSIMSEQKKAMKDILNDIDDILPLDLFSTETFKDELADANDKRKKTLEKLDALDEDLKTEYALSEPNEQFIKSDFQKLQEATGKGKNATPIHYNAKAYRESDIHKKKGDIETRTEAYLKIKKEEAKEREIEKLKERLKNYDYADADEFYEMAKTIGYENLTAEQQRYFTQIENTRELEAGFKGVAVGLYDSGKDAVVGLWDMVTDPGGTVEAITGAMAHPIKTYEAISAAIEESYQKDMVNGDTYSRARWVSYAVGTVVTSIVGTKGVGAVSKTGTAAKVTTKVKTAASKSATAQKAITVSKQTVDHIKQKVNTGIEVSKKHVKTKLNQIGDLTLADILPYHPRHDLVPAGVPYNAVNGVTLKEGLQKFAKVILPKPYGTSSSGRRTPAPHVPPVTVKYGEHYAKWSRKKVLKPNVEYKTKEGYTYNTDNYGRITKVEADLQLGEAKRNQYAQSNAGKPQDRLPDDDGGHLIGSQFRGSGELDNLVAQNSQINRSGGEWYKMETEWAAALKEEPPRKVSVRIRPKYLGDSLRPDSFEVIYRIEGKGLFKKFIKNQAGG

SEQ ID NO: 95 - protein, 112 aa, Bacillus subtilis
  >ABP11825
MDKDFLIIKIKDIQKGDTLTNRACGNWDMKLSRAKECKRAIVVRSGVILNVYKIVDAWESDEPAKITKTNNRVRFQLAECRDYSYLIGGTLKTKTQNPVSSLSLETLMELVK

SEQ ID NO: 96 - protein, 306 aa, Bacillus subtilis
  >ABP11826
MYLYKVNNQNQIEDIREKPFKKEKEIQDLCEANLQQMLGLGFVKSEFRISNFRIDTLAFDAETKSFVIIEYKNTKNFSVVDQGYAYLAAMLNHKADFILEYNENHDLPLKRDDVDWSQSKVIFISPVFTVYQKQSIHFKDLPIELWEVKRYENDLIQLNQMKADGVSESIKTISQQSETIQEVSKEIKVFSEEDHLADKPFDIIELYQQLKEFIFNLDDHISIKPTKLYIAFTSNKRNFTDILLLKSGLKLWVNMKKGELHDPEERMRDVSETGHWGNGDYEIFIKDEENIEYIMGLIKQSYEKNK

SEQ ID NO: 97 - protein, 335 aa, Bacillus subtilis
  >ABP11827
MKKRFILLGLFASVFMLAVYISFQNKNTHPVQSPVIHPEEDRIFFIYSNLFIKESVLLSTSTGERFNRRTFKVADVPYIQMKSYKSTDLVLLAEHEPFYYTLEKDAIKEHPLSDPFAFWHEGKDVSVKAYNVDTTGNEIRINDKKMKKEYTLTLPSLVTMGASDENYIYIIQSMAIYVIDRKTEEMIETLSLASYADQFADSKEFIVASSEHELTVIEKGTWKATYIAYPEDLEYADTVYYDKESGSFYVTYEDKKGEANLLEYGKEFSFHTYSLNFPYMEAKFKGNLLYIVAQEEHKKGIGGYVGVFDIHSKKMLYQFDLPEEQVKVQDFVVVD

SEQ ID NO: 98 - protein, 284 aa, Bacillus subtilis
  >ABP11828
MGGSYLSDLCSMYQKDKFFTGFVPDELLTYACELFPLSEKETVTALLNCSMGNKAKSFVMFTSKGLYWKRFGEQEGCVTWEAFTDIQSIKSTDDYEIWFEGEEVFDVGFSSYPADLLAELLRMIQQFLSENGSDLLTEAWRDHVSVSASELKEISTLFQNSHDKMFGLTNGLLVGNEISEKREVRLRKRLHIPKDQEMISFWSTFPVKQTDGITLTDKGIYFSDPFLRLFYPWHVFKETPVMLKDQELIVGKENVIQLLENLMPAEDVFAFIEQVKRRISAVTS

SEQ ID NO: 99 - protein, 298 aa, Bacillus subtilis
  >ABP11889
MLRKKGQETKDYKTQQVESWGLRLIGKNEKIEKKSNISIAILDSGIDSNHEDLKGVVKKEYNALEPSKGVIEDKFGHGTAVAGIIASNDNKIGTLGIAPYADIYSVKVLDDKGRGSVESIVKGIEWSIDNNVDIVNISVGLKKSDQKLKRVIDEANEKGVIVVAAAGNNYGLNADYPARYQNVISVGAINKKMKRAKYSARGKIDFVAPGEDILTTSPKDNYINVSGTSMATPFVSGVIANIIMQEPVKYSKTKSRFTSIYKTLKKYSTPYLSEKSDMKSLGNGLISLKKETNNEKIN

SEQ ID NO: 100 - protein, 308 aa, Bacillus subtilis
  >ABP11890
MKKSIKFIAISLIFAIIVSIIPEKNVASAGAETPVEITNEDLQRALVENGDIVDPDSVEIVKNNEDTIKAEVDVQTDDFGIDQDLDGSDSESLIDEDLDESSSETVTAEVDKEDATAIVTSVEKDEDGKDIEKKYEVDIEEADGDDIVATFKDLDTNQVYDVNTKEAQASFAFLVPIAVVVGGALVEHLVAASLAIVIAGVTYTVATKVRSKLKKKKKYYYYAATLNKNKTNMYIGPALSKKQAVSRLRKGDVWSVSKSKAKNVAQTAGGGRKPVGPEIHNKKDGKIKKGTYYYHYHTYNRKGGHSFY

SEQ ID NO: 101 - protein, 52 aa, Bacillus subtilis
  >ABP11891
MWESIQNGKRVNKIFESKDGNYISNFTVQGNVEKIEKELVFIRGILEKEKNN

SEQ ID NO: 102 - protein, 153 aa, Bacillus subtilis
  >ABP12521
MKLIYPYGADKIYLGNPVELFRDQDTGDYIIPKNATDIPPELNGEGMWRPMFNEEKQTWIETADQAYKKSLLEDVPSESNPTNDQLSALGKQLTEEKLARIQADQAQKALGMQLTEEVIARKEAEALSQSLGKQIAALKLDLLNLKGGMTSES

SEQ ID NO: 103 - protein, 63 aa, Bacillus subtilis
  >ABP12522
MSLNFWVYALFYKWATTSMVREAMMFHDCSVDDLKEGVSEKYVTLAQFKEITDQTYEETMKAN

SEQ ID NO: 104 - protein, 92 aa, Bacillus subtilis
  >ABP12523
MSELSEVPDMNLLEKEITEIKTEQKTLEQRVSVLERSSDRQDQQIMTLNEKLNKIEENTTWIKRTITGAIITAVSTGIIGGAIAIMYSLLQH

SEQ ID NO: 105 - protein, 250 aa, Bacillus subtilis
  >ABP12651
MKLEQQEINILHSDSGPYGIAISPEGKVWFTQHKANKISCLDRTGQIQEYIVPTPDAGVMCLTVSSEGDIWFTENRANKIGKLTAKRQFIEYPLPHQHSAPYGITEGPDGDIWFTEMNGNRIGKLTSEGKIHEYELPNEGSYPSFITLGSDHSLWFTENQNNAIGKITESGELTEFPIPTPAAGPVGITKGHDDALWFVEIVGNKIGKITVSGDITEYDIPTPNARPHAIAAGVKSDLWFTEWGGIKSEG

SEQ ID NO: 106 - protein, 58 aa, Bacillus subtilis
  >ABP12652
MVYRMGGNKIGRLTSDQTIEEYTINTPHAEPHGIGCDNDGTVWFALECNKIGKLKLTK

SEQ ID NO: 107 - protein, 43 aa, Bacillus subtilis
  >ABP12653
MKVKEKRIVVNKFPSQPDEEDCRNLTLLGWGSGGFFLFLHTFR

SEQ ID NO: 108 - protein, 49 aa, Bacillus subtilis
  >ABP13703
MKQRKRIIQKDRRKLLKYFNAKFTAEERAMESLFCEKTSQSSSNVLLND

SEQ ID NO: 109 - protein, 185 aa, Bacillus subtilis
  >ABP13704
MKTKSEPKVILEPAKESDLPEFQKKLQEAFAIAVIETFGDCEDGPIPSDNDVQESFNAPGAVVYHILQDGKNVGGAVVRINSQTNHNSLDLFYVSPEYHSQGIGLSAWKAIEAQYPDTVLWETVTPYFEKRNINFYVNKCGFHIVEFYNEHHSDPHIHRNGRVDDKPLPDNDDFFRFVKIMKKKD

SEQ ID NO: 110 - protein, 44 aa, Bacillus subtilis
  >ABP13705
MPLTLIWRNFEFSEKFLGTYADNVLKVLQEAQEELEDEFKIIVE

SEQ ID NO: 111 - protein, 303 aa, Bacillus subtilis
  >ABP13706
MSLEEQLQSKEEELTKLVSTFAAKEGTNETSISGLEFIRSAKPLMPVHTMHEPALCIVLQGRKVISIIGEDFFYGKGEYLVVAVDLPVIGEILKASEREPYLCLRLNFNLMQIAEVSKEYQQHSTNHNAAGRGIFVDQTDGVILDALIRLVKLLHTPEDTEILAPLIIKEILYRIMQGKHGHTVKSLVAKGSKLSEVAAALDYLRNHFSQEIKIDALAKKVNLSPSALYHHFKQVTMMTPIQYQRALRLHEARRLIFGKDMRVADAAFQVGYESPSYFNREYRKMFGKPPGKDRKENLNLYYV

SEQ ID NO: 112 - protein, 82 aa, Bacillus subtilis
  >ABP13707
MEKNNHSYGGLWVTKDRYIRHELLSNGRYVEARGNVECAYTGNYQITGDRIEYQDDAGFTADGDFINGILYHAGMVLHRDRS

SEQ ID NO: 113 - protein, 243 aa, Bacillus subtilis
  >ABP13708
MSIKNKVVLVTGGSSGIGAATVDLLAENGATVIAAARRTDRLETLVTTLQQKGYHADYKQLDVTDFGQMQQTVQEVTDAYGKIDVIVNNAGVMPLSKLDSLKIAEWNRMIDVNIRGVLHGIGAVLPVMKEQNSGHIVNIASIGAYEVTPTAAVYCATKYAVRAITEGLRQEATHNIRTTLIAPGVTESELADHITDKQASEAMIEYRRQALPASAIAHAILYAISQPIEIDVSELIVRPTLSL

SEQ ID NO: 114 - protein, 260 aa, Bacillus subtilis
  >ABP13709
MRRIDFGLTFLICTLIMLFNEIWKLLGNRPEAFKYGSIIYQVIAVFSSIITNVAIGVAGAISFYYIAQLIDKKKNRELYTDLRKHLLFMFYNHLKLLTRLDQFREVNNRERRVADFYDIFDIPVFYDNFKKINSKEEVTRFKKNLYDYFATQSEQQIKVFTEAFEKDIKKLKEKSNIRFFKESKDLIDTVCIIYDDDFSMISSIYLSNFEDTQNKSNYIEELVKDYYDFLNATVILYEELEEFLESMDKNRWVVFIKMLD

SEQ ID NO: 115 - protein, 48 aa, Bacillus subtilis
  >ABP13710
MENAQEIYELVKEMSKTVKEIDETTKRIENTTKRIAKGYELITEELAE

SEQ ID NO: 116 - protein, 339 aa, Bacillus subtilis
  >ABP13711
MTYRVGSMFAGIGGTCLGFIQAGAEIVWANEIDANACITYRNYFGDTYLQEGDITQIDKSTIPELDILIGGFPCQAFSIAGYRKGFEDDRGNVFFQILEVLEAQRNVYGRLPQAIMLENVKNLFTHDKGNTFRVIKEALEAYGYTVKAEVLNSMEYGNVPQNRERIYIVGFQDENQAEMFRFPEPIPLTNQLNDVVDRTRRYDERYYYDETSQYYEMLREAMVSTDTTYQLRRIYVRENRSNVCPTLTANMGTGGHNVPLVLDYENNIRKLTPEECLLLQGFPADYHYPEGMANSHKYKQAGNSVTVPVIRRIATNIINVLNGETNANDEQEHQYAITQ

SEQ ID NO: 117 - protein, 78 aa, Bacillus subtilis
  >ABP13712
MIPFLGNRIQNAREARGLKPSQVADKVKVTRSTYSLYESENRTPSLETFIRIAETLNVSADYLLGLKEEMTSLNEEEN

SEQ ID NO: 118 - protein, 382 aa, Bacillus subtilis
  >ABP13713
MFFTNQPASNRTTYKQMLSSTGSLSNLFSESDSPYLVSRNVENAFCEALGAENLGRSDCSADASKDRVGIGIKTFLHGNGHTLQKVAEFNRDSDLYRGKSPKELINIVATLRNERIEFTKRTYGIDTMIYHCVTRKPGKILIFEEPMDLVQISSITNIKVSNNRNTITFEDGLHEYSFNVTKSTLYKRFITDEPIEEIDVEILENPYQELAKLFGFEIAPIQVPEVSSPIENFEYVILPLFSDRGNKRHVPEKSGLNQWNAAGRPRNANEIYIPIPMWIHRKFPEFFPARDKPFQLRLPDKSLLSAKVCQDNSKALMSNPNSALGEWLLRQVMNLGERELLTYEMLERLSIDSVIVYKHSEQHYSIDFREIGSYDEFENENN

SEQ ID NO: 119 - protein, 141 aa, Bacillus subtilis
  >ABP13714
MTDTFSKEQRRKNMQAIKSRSKLEDKVTKELWNRGIRFRKNVKGLFGKPDIAIKKHKIVIFIDSCFWHACEKHGNKPKSNTEYWEKKLQRNKERDREVNKYYEEKGWNIKRIWEHELKEDFDETINRIIAFIEAVKHEQRK

SEQ ID NO: 120 - protein, 49 aa, Bacillus subtilis
  >ABP13715
MLKIKKLDFMPFFNRMICFVDVKNPDEADKKALAKDILENNKDQYQGYD

SEQ ID NO: 121 - protein, 224 aa, Bacillus subtilis
  >ABP13716
MKFIELDPALQIKVRQLEANAEEHQDKSHPDVRALWLELQKEDSICGALSEKDGSYKVCLRAPVEERNRCSLHGGKTLKGEQMTPAQKLNMMKNLRPRVVEHCWYAEESNFLASLTESEIKYMSFLEKSVKDQYHVNDGLEELLLEDILQSAIIHMRMVNRGVFEKGSRHTARPLQEVLKTIKELGWTCKEKGGKVQFVSVRNDFMASIFGNNTEEEEEDKKLN

SEQ ID NO: 122 - protein, 58 aa, Bacillus subtilis
  >ABP13717
MSLKEKLAELNKRAGKLEGSLKKASKKASSEADRLKKKRQEREYYDAYEKKFPIDKNF

SEQ ID NO: 123 - protein, 50 aa, Bacillus subtilis
  >ABP13718
MKKDWFSQRLELINKEQKLNEEFNLWKLQQITKRMKEVTKKLDELETERV

SEQ ID NO: 124 - protein, 192 aa, Bacillus subtilis
  >ABP13719
MGLFNKKSEMVKFEEELNVVQGSIREVEAELRDFDTSKKGIELELKLGADSSLTKRLKKVSEKVAETEKCLAELRQREGEINAEKRTAYLNELADKDLASIDKGRRATVIKYELQALMRVVDERDGRWGYSKPENLLKEYGIEIGHIPAEHLRREEFDSFWKTRKNDAEKRIQNECQEAIETLKKYLGGFDK

SEQ ID NO: 125 - protein, 209 aa, Bacillus subtilis
  >ABP13720
MESKVNMLRILEFYMGETGNFKKLVVIQEIYRNNPSKMKGCELSFLKDNKFVAKGFFEAETIMVRNSFHSYNSELPELKEHHFKKMEKRDQDSHYPVSETTVLYLSGYVFAEFKFHKIANDKKIGDKVYLPIKLDDKQKPDSNEFCKLLVLEEYRDGTFELPELPKRAEMFTCWVRLELAPDSKNDSGVKVSEREFNKARMGEIKGNIA

SEQ ID NO: 126 - protein, 273 aa, Bacillus subtilis
  >ABP13721
MSEDVKKYFTTGEFSKLCRVKKQTLFHYDEIGLFSPEIKKENGYRYYSYHQFEIFQVISLFKELGVPLKEIKCLIKGKTPDKILHVLKEKSIEIDKKINELKQLQTILQTKVTLTEQALETDFSSISFEYLNEETFMLSRKTLNLPERKYVAAISELIHEVQQYELDEGYPIGGIFAREQILEKDFYNYSYFYIKVKDGAENINYHVRPKGLYAVGYEIGGKTEEAYRRIIEFIERNGMQIGENAYEEYMLDEMVVDGYENTYAKILLQVKEV

SEQ ID NO: 127 - protein, 419 aa, Bacillus subtilis
  >ABP22957
MREKKLGPVLLSGLIVGPILGSGIILLPPIIYGKTGDYAILAWFIMMIISFLFASLFGKLSVLFPNESGVAHTVELAFGQHIKQLTSVFFIIAGSVGPVAVLMTASQYLKALFKSNGWSLETYGIILMMICLFVLLSNISSVGKVSFMFSTVSTVVLLSGGISSIPFMRDKAFIKTPFHLDDFGYSILLLFWALVGWEIIGNYSLDVKNRKRTIPQAIVISSVVITTVCIVVAAAYQWIDLHHTHTLTIILIPLLGTSFASPTMAFITTILCMSTYLLVTGGVSRLIASENKKITLISYRSKTNIPIGAISILTLVHAIVFILLFINIINVEQIVGMANAFFISNAICGILSAYKLLPGKFSKSLSLMLIISFLIILSFSSIWILLMIALITTFYLIRHFIWIRQLKKSATNSQDKLRF

SEQ ID NO: 128 - protein, 299 aa, Bacillus subtilis
  >ABP22958
MEIRHLKTFITIVEKGGFTKAAEYLGYAQSTITSHIKDIEQEIGGPLFNRFGKKMLLTEVGEYLLPYANEMIRISEKVKQIQSNDEPMGNLVIGAPESLTVYRLPPIIHEFKKLFPKVKITLKSSTCWELKDDLRNGKVDLAFLLEYEQEEADLYIEKLITEPMILVFPKQHKLQNTPFDDFYFSSDEVILYTEHGCSYRTYFEEYMKHQGLVSENTFEFWSVEAIKQCVMCGLGISLLPLITVQKELKENKLSGLIMDETRIITQVAYHKKRWNSLAMAEFINIVKKHAELWKRTQTL

SEQ ID NO: 129 - protein, 187 aa, Bacillus subtilis
  >ABP22959
MNPLLLDVPLQLETERLILRAPHQTGDGKIVNQAIRDSFSELKAWLPFAQELPTVEETEINLRNAHINFLKRESFRFLIFDKDSNDFIGITSLQRIDWNIPKCEIGYWVNTKYSGNGYMTEAVKKLANFGLHNIKFRRIEIRCDSTNLKSRAIPEKLGFVFEGTLRNDDLSADGSKLTDTCFYSIVK

SEQ ID NO: 130 - protein, 102 aa, Bacillus subtilis
  >ABP22960
MVDQLWAYFLNLIEEAIETGKSETYFPDQPLLLKMKSISNDMLLFEIDQKQKVLLPKLDFFESLLKNAKSFFETMNFVLEGNCDYEYELNKIDELQTKIKCM

SEQ ID NO: 131 - protein, 573 aa, Bacillus subtilis
  >ABP22961
MKVFEAKSLLSEAENRAKDYKELKNQMIKLRKAFKAVADLDDSEFSGKGANNIKAFYHDHVGVTDQWIDLIEMKIAFLTSISGVLEDASLSDAYIEESFLEHELTNAYKKSKSIMSEQKKAMKDILNDIDDILTLDLFSTETFKDELSSAENKRKKTVDKIGDVDENLKTEYAITEPNEQFIKADFQKLQESTGKGKNATPLHYNAKAYRESDIHKKKGDIEKQSEAYLKIKKEEANKCEIKDLKKQLVKVTDPDEYLKIAKKIGYENLEPEQQVYFRQLEELQQKAEIGKGIAMGMYEAGKDTVMGLYQLARHPIESLSGTVNAALHPIDTYKIIAKDIEDTFQREMINGDSHSRAKWVSYVGSTVVLAIVGPKGIDKVSKVAKAGSKVAALKTLEVSKTGIKKGIEYVKIPSVFEQQFAMAGGSGTFPFNVLDGENYKNSALEIFKNSSTVQGLKKAKPHEVVNELKTFQSRKYTFGGQSFLIDKRGMKHILERHHPNLWDGSIKSQQSFLNKEMTVNDVADAIESIMKQNREELTKKGTKFSYQIRGSYEGQQYVVGFQKGRVGQFYPEK

SEQ ID NO: 132 - protein, 84 aa, Bacillus subtilis
  >ABP22962
MVQEVMVMKKDFGDSISNKVYEYRVLARLSQQELAKKVGVSKQTIFVMEKGNYVPTLLLAFRIAEFFKVDVNEIFTYEKGNDQK

SEQ ID NO: 133 - protein, 58 aa, Bacillus subtilis
  >ABP22963
MNNKKNIFDIVMYIIFGVLSLFLVAKTDYGTGVLVFVAILYLAVIAYKIKQVFSNSDS

SEQ ID NO: 134 - protein, 222 aa, Bacillus subtilis
  >ABP22964
MRKKRVITCVMAASLTLGSLLPAGYASAKEDSKTTPSYEELALHYKMKSEKISSNGKLVEIEYVSGNETHKVQMNGNNHTVKVDGIEQKGLNFEYDENVAKRTNYENNNLKSNEFTTQAAKPKKGYHYVGTLSGHTKAAKNALSVTMSLVGIVPGLGWGSKAATILFSYWAKEQIPDAYYKYDLYEKGAMTDSWYQYATVQFLKIKLIKRKWANLGQVLLQK

SEQ ID NO: 135 - protein, 87 aa, Bacillus subtilis
  >ABP23145
MKNFDKGTVVRTVLLLIALINQTMLMFGKSPLDITDVQVNQLADALYTAGSLIFTIGTTLAAWFKNNYVTAKGHKQKAILKQNNLTK

SEQ ID NO: 136 - protein, 273 aa, Bacillus subtilis
  >ABP23146
MTIAVKKNLVSEAKYALKCPNPMTAEYITIHNTYNDASAANEVSYMIGNTSSTSFHFAVDDKEVRQGIPTDRNAWHTGDGTNGPGNRKSIGVEICYSKSGGAKYYAAEKLAIKFVAQLLKERGWGIDRVRKHQDWSGKYCPHRILSEGRWNEVKAAIDAELKALGGKSSSKKTTSSKAVKKPSSSKKKSSFNLPSGIFKVKSPLMHSAAVEQIQTALAALHFYPDKKAKNFGIDSYYGPKTADAVRRFQLMNGLKADGIYGPATKAKLEALLK

SEQ ID NO: 137 - protein, 52 aa, Bacillus subtilis
  >ABP23147
MKRKQTFIFSMILLSVASIGLRSFWTNPFTTGVMIFVLALTIYAIIKDLRRR

SEQ ID NO: 138 - protein, 81 aa, Bacillus subtilis
  >ABP23148
MEYHLKSRQEVEDFIRHEVLTTKEAAELLGVNRQRVSQLISSGKLNPIKKLSGISLFLRTDLEEKKKELEAGRKKYRPYDE

SEQ ID NO: 139 - protein, 306 aa, Bacillus subtilis
  >ABP23149
MDEGTYNIDIVGFHGTSLESAQKIITEQNFTSGDIRNDHWLGQGAYFFREDPEQAKIWAKNKIKGSETAVIKTIVSLDNNSFLNLDTRSGLNYFNRYIKTEVKRKILEEKAEIELTTDDHSKIKHIYRCFFCNELPTNIKAIQRTFFVQSTLNEDETFKKMDVFVQGVQVCIRDLSVIDFTKTGINNVINMHTFRRRKKTKQKENYRKDVMKMRREFNNPELIKDAENLGIKITLNSSEPGVFANVNGERYRINIDDLFSECDDDLYYHEDFKLDDFSITRDSNQHKVEIIKEEKNFYKNELVEAA

SEQ ID NO: 140 - protein, 60 aa, Bacillus subtilis
  >ABP23150
MKSFFQFDDYNIIDVNYKFNNNFEGDEAVLSPIFDFELEFEDETKDEADLILGIELGIRI

SEQ ID NO: 141 - protein, 62 aa, Bacillus subtilis
  >ABP23151
MTDFERKVYQIIVNMHLYGKNPTLDDLKRKTGKSKEDIRTAVKSLLMEGELKWDKQQKKWII

SEQ ID NO: 142 - protein, 973 aa, Bacillus subtilis
  >ABP23223
MTDSWQNGFIEKINRNGNNGGLRKPQYGALSAIRAHWTISSKPATIVLPTGTGKTETMLATILSEQIESVLIIVPSNLLRDQTFEKAKSFGILPDLKMVGKNILYPNTVLYKTRIKDETEVWEWFSEANVIVSTVNAVNGLSTSILNKLVEKVDVLMIDEAHHIAAGGWSSLREKFLNKRILQFTATPFRADGKKIDGDIIYNYSLSLAQKDGYFKPIDFYPIEEFNEELGDIQIAEKAVELLNKDLEDKYMHQLLVRANSKKRAEELYNKIYSIYKKFNPVLIISGQSKKNKENLKKLREGIAKIVVCVDMFGEGIDIPNLKIAAIHDKYKSLPITLQFIGRFARSKSGIGNARIVTNIANDDLKDALQSLYSQDADWNQLLSMHSSDAIQTEISHRKFINQFYSNDNINIDISQIKMRISTRVFYLGGVHWNRKGWRSVLNVDKTEFFINEESSVMILIESIESQVDWSDQKDISKYNYDVFIIYVDKKNKLIFINETNASKGNQLIKYMFSEANQISGERVFRVLDGINQLMIGTLGLKEQPSGRISFRMFAGTNIKDGINQVARASTTKSNLFATGYKDNNKISIGCSYKGKVWMRWVDSVVFWRKWCQKIGSQILDSSINTDYILENSLQSEEITEYPRGIPYKIQMPVEFELSNSELKAFYIPNEDKEIPFYLCEFNNPRLDGKQLLFELWINERKYTFSQTLKERGFVINRILGKDIKIKKSRNMITVEEYLQDNLPQVTFFNEDGSLSIVEGNLVVNKKPLAEVLFPKEKLHIVDWKKLKVDITIESQGLTKLNNSIQYASIKNIVPVDSLIIFDDDNSGEIADIVCISTNEEHRKITVQLYHCKYSHGTNPGARLLDLYEVCGQAERSITWNDSMVELLKRMRFRENKRINENKTSRFEKGNLSDLKTIENQIRSGFETEMKISIVQPGVSISNISQQMNQLLLATDTYLKETYGIDLNCYFSK

SEQ ID NO: 143 - protein, 376 aa, Bacillus subtilis
  >ABP23238
MSQAIPSSRVGVKINEWYKMIRQFSVPDAEILKAEVEQDIQQMEEDQDLLIYYSLMCFRHQLMLDYLEPGKTYGNRPTVTELLETIETPQKKLTGLLKYYSLFFRGMYEFDQKEYVEAIGYYREAEKELPFVSDDIEKAEFHFKVAEAYYHMKQTHVSMYHILQALDIYQNHPLYSIRTIQSLFVIAGNYDDFKHYDKALPHLEAALELAMDIQNDRFIAISLLNIANSYDRSGDDQMAVEHFQKAAKVSREKVPDLLPKVLFGLCWTLCKAGQTQKAFQFIEEGLDHITARSHKFYKELFLFLQAVYKETVDERKIHDLLSYFEKKNLHAYIEACARSAAAVFESSCHFEQAAAFYRKVLKAQEDILKGECLYAY

SEQ ID NO: 144 - protein, 200 aa, Bacillus subtilis
  >ABP23224
MSKIPPEKYYEACITYHLVNYFEFTLEKKIYPFSISQIEEKKEGYDFGYKMSEKSFFIQYKRPYKVIPKDTYHWKIEIEQLKTINRKANNINTYYALPSFGDSMGWYEALDNTFFVNSRSLEYQIKQINRGRNIKTTFISPEKILLDKFYRISCNIVGDLHSVAVSQKNINSKIGNITNYIKGLNEDVKSSTWLYILEED

SEQ ID NO: 145 - protein, 623 aa, Bacillus subtilis
  >ABP23225
MKYENVEVLGSYSVREGGSINFSMGKNLELGTEINTYIHELFHMHLTNYSSLGFLLLLFEKECNLSLEYQDELHYNQIKELSTIIFNRTVDVQEVYANNQELLWLENNINSEFKEKSFKLKPKKYQEYCNKLNIITNDMRLNNEEKRYWIDRVCFYALNIQIFSDKFIEALKSRQKLSEYLSRNHPNKRLDEALVKYSKNEKFDGVVEIRIQDILSKIKKINIIKYFNEILSQLEPNATNFKIGDYLCENDIKKFIELNQKRMDERVKLFDFYNLDVIKVDDISNHLNFGIFAIKNYESTINKENFYYITEALINLTPSYISEEVSYDFLNNPKIKVIGIPSQEFDIAKMKPNYIEVKDTPIVVLIDSYNTAKKILKVLLNGELYVGDLYEQTVKNFSTILFFRERTEPKIIYIFPTLKKMSIRLVKELGIEDILVYSKDTRFKKILSIFNCEVEMLKFIKWIFSFIMKSSCIFTSIGDPATKMSFNLTRSLFDDVMKIKIPNYYIHWAALPTKKTIGEPFYSLMEFENGENIGSFKATNQNTIIFFLNKNDAVNYRKKIFTTDSMAHKLEVVGIDRHYWNIIEKYILETGINICICTDVNNNIGKIMKLKEVDNIITQFSKV

SEQ ID NO: 146 - protein, 65 aa, Bacillus subtilis
  >ABP23226
MKFKLTLCAVIALIGVSFISSSLGNEVNVASRNMTSKAANDSTNSLADKAIFDKEMTIAENGTLG

SEQ ID NO: 147 - protein, 378 aa, Bacillus subtilis
  >ABP23227
MRSLGTISSPHVGMKINEWNRHIQKFNVTDAEMLKAEIERDIDIMEEDQDLLIYYQLIAFRHQLMIDYVIPTEGNQMELSEYLKRIEGSNRKMEKLVEYYYYFFQGMYEFKEGNFLSAITFYQKAENTIPYISDEIERAEFYFKMAEVFYHMKQTHVSMHYSSQAYNIYKTHDLYSVRRIQCHFVIAGNYDDLESHEKALPHLEQALKGARLLESKNKRIYGQALFNIGNCYLKMGELTKAAKYMEKSIFQFKKSNFNNLTQAYHDLALIYFLQHKQEQAMDCFRKGVRFACKFDDDLFKIMFEGLQTLFIKKGEASILLNVFNKLETSQGYPYMEELALLAAKFYTEIGQMDDSVICFKKMVHARKQIQRGDCLYEI

SEQ ID NO: 148 - protein, 107 aa, Bacillus subtilis
  >ABP23228
MTVREELIKRNPTPIMKNILKRYEEAKEFIQHSTKEQFEEDLSRVKNKLDTLTRAYLESANDYMNPMLREMYKTEKLLKEYDETASVVITAIQSSKVEIVLPSQNQI

SEQ ID NO: 149 - protein, 130 aa, Bacillus subtilis
  >ABP23229
MDLFEECIEALKDPKEILSDELTEQYFETLNNKFPITSWARIDWDKVPQKESIETYDDLYNWLKFQGIVDTTINLLWNPSDVPVVRTTLENALEVLDDVLAVGSDTFMYSDHGFVIEFFHDGEVTIGRSE

SEQ ID NO: 150 - protein, 51 aa, Bacillus subtilis
  >ABP23230
MAQLFTAGLFLFQIGLAIMETEKGLLYKKSAEQFNNLLLLNEIRLTYTLKF

SEQ ID NO: 151 - protein, 156 aa, Bacillus subtilis
  >ABP23231
METEKMGQLYQQIAEQLNEMIPSEWTKIVLYAEILDDSSEVYFFFNTPQSEEYIYSHDIPKQFDVSKKIYVSLLIELQELFEELREEFKANNQDTWTNLTLKLENTGKFSIDYDYTDVIASDLNGTQRQVVWEYKNLGILPEDKEDKDFVINYFSL

SEQ ID NO: 152 - protein, 670 aa, Bacillus subtilis
  >ABP23232
MVMKVFEAKTLLSEATDRAKEYKELRTQMVNLRKALKGVADLSDSEFSGKGASNIKAFYHDHVGVADQWIDYIDMKIAFFNSIAGAAEDKGLSDAYIEESFLEHELANANKKSKSIMSEQKKAMKDILNDIDDILPLDLFSTETFKDELADANDKRKKTLEKLDALDEDLKTEYALSEPNEQFIKSDFQKLQEATGKGKNATPIHYNAKAYRESDIHKKKGDIEKRTEAYLKIKKEEAKEREIEKLKERLKNYDYADADEFYEMAKTIGYENLTAEQQRYFTQIENTRELEAGFKGVAVGLYDSGKDAVVGLWDMVTDPGGTVEAITGAMAHPIKTYEAISAAIEESYQKDMVNGDTYSRARWVSYAVGTVVTSIVGTKGVGAVSKTGTAAKVTTKVKTAASKSATAQKAITVSKQTVDHIKQKVNTGIEVSKKHVKTKLNQIGDLTLADILPYHPRHDLVPAGVPYNAVNGVTLKEGLQKFAKVILPKPYGTSSSGRRTPAPHVPPVTVKYGEHFARWSRKKVLKPNIIYKTKEGYTYTTDNYGRITSVKADLQLGEAKRNQYAQTNAGKPQDRKPDDDGGHLIATQFKGSGQFDNIVPMNSQINRSGGKWYEMEQEWAKALKEEPPKRVNVNIESIYKGDSLRPTKFIIEYTIGNKTKFVTIKNQAGG

SEQ ID NO: 153 - protein, 112 aa, Bacillus subtilis; identical to SEQ ID NO: 95
  >ABP23233

SEQ ID NO: 154 - protein, 306 aa, Bacillus subtilis
  >ABP23234
MYLYKVNNQNQIEDIREKPFKKEKEIQDLCEANLQQMLGLGFVKSEFRISNFRIDTLAFDAETKSFVIIEYKNTKNFSVVDQGYAYLAAMLNHKADFILEYNENHDLPLKRDDVDWSQSKVIFISPVFTVYQKQSIHFKDLPIELWEIKRYENDLIQLNQMKADGVSESIKTISRQSETIQEVSKEIKVFSEEDHLADKPFDIIELYQQLKEFIFNLDDHISIKPTKLYIAFTSSKRNFVDILLLKSGLKVWVNMKKGELHDPEEKMRDVSETGHWGNGDYEIFIKDDEHIEYIMGLIKQSYEKNK

SEQ ID NO: 155 - protein, 273 aa, Bacillus subtilis
  >ABP23235
MKKRFILLGLFASVFMLAVYISFQNKNTHPVQSPVIHPEEDRIFFIYSNPFIKESTLLSTSTGERFNRRTFKVADVPFIQTKSYKSTDIVLLAEHEPFYYTLKKDVIKEHPLSDPFAFWYEGKDVSVKAYNVDTTGNEIRINDKKMKKEYTLTLPSLVTMGASDENYIYIIQSMSIYVIDRKTEEMIETLSLASYADQFADSKEFIVASSEHELTVIEKETWKATYIAYPEDLEYADTVYYDKESGSFYVTYEDKEGEANLLEYGKEFFIHIV

SEQ ID NO: 156 - protein, 47 aa, Bacillus subtilis
  >ABP23236
MYIVAQEEHKQGIGGYVGVFDIHSKKMLYQFDLPEEQVKVQDFVVVD

SEQ ID NO: 157 - protein, 285 aa, Bacillus subtilis
  >ABP23237
MGGLYLSDLCSMYQKDKFFTGFVPEELLTYAYELFPSSEKETVTALLNCSMGSKAKSFVMFTSKGLYWKRFGEQEGCVTWEAFTDIQSIKSTDDYEIWFDGVEVFDVGFSSYPADLLAELLRIIQQSLSENGLDLLTEPRIDHVSVSASELREISILFQNKHDKMFGLTNGLLVGNEISEKREVRLRKRLHIPKDQEMISFWSTFPVKQTDGITLTDKGIYFSDPFLRLFYPWHVFKETPVMLKDQELIVGKKNVIQLLENLMPAKDVFAFLEQVKRRISAVTSS

SEQ ID NO: 158 - protein, 37 aa, Bacillus subtilis
  >ABP23502
MFVLLLYPKQSLLIHYSSKAEKGRTLFILFLASTLNI

SEQ ID NO: 159 - protein, 41 aa, Bacillus subtilis
  >ABP24563
MFNGKHLKVKACFKSNAFLIIIKESVYIFISPLPDDAFRTP

SEQ ID NO: 160 - protein, 484 aa, Bacillus subtilis
  >ABP24564
MDQREKMDTAGGNTSCKHKKFFRKITIISTFGGLLFGYDTGVINGALPFMAQRDQLDLTPFTEGLITSSLLFGAAFGSLAGGRLADRIGRRKTILNLAFLFFIATIGCSFAPNTSVMIICRSLLGLAVGAASVTVPAFLAEMSPAEQRGKTITQNDLMIILGQLLAFTCNAVIGTSMGEYAHVWRFMLILATLPAIFLWFGMLIVPESPRWLASKGKVGEAFRVLKHVREENCAKAELTEIKASINRETEINRATLKDLSVPWIRRLVGLGIGIAVVQQITGVNSIMFYGTQILQKAGFARDAALVANIGNGVISVIACTFGIWIVGKVGRRPLLLTGLAGTTASILLIAICSITLQGTPVLPFIVIGLTITFLAFQQSAVSVVTWLMISEIFPLRLRGLGMGISVFFLWMMNFLIGLTFPVLLDQLGMSSTFFVFVVLGASAILYVKKYLPETKGRTLEELENDFRSNQGVRKASSGKGEINM

SEQ ID NO: 161 - protein, 388 aa, Bacillus subtilis
  >ABP24565
MINGEKKVDRPIRWAMVGGGRGSQIGYIHRSAALRDHHFQLVAGAFDINPERGKDFGMNLHVTPERCYLDFQQMFEEEAKREDGIEAVSIATPNGTHYEICKAALNVGLHVVCEKPLCFTFEEAKELENLAKKKNRVVGITYGYSGHQMIEQARQMIANGELGDIRIINMQFAHGFHSDPVEMNNPSTKWRVDPKFAGPSYVLGDLGTHPLFLSEIMIPELKINKLLCTRQSFVKSRAPLEDNAYTIMEYDNGAVGTVWSSCVNAGSMHGQKIRVIGSKASIEWWDEQPNQLRFEIQGKPVQILERGMGYLYPEALQDDRIGGGHPEGLFEAWSNLYSRFAVAMEAADRGKELEHMWYPGIEAGVGGVRWVENCVRSADKGAVWVDYQ

SEQ ID NO: 162 - protein, 309 aa, Bacillus subtilis
  >ABP24566
MSIHIAGAPCCWGVDDPKNPYLPPWERVLQEASQAGYKGIELGPYGYIPMDIERVQAELLKNNLSIIAGTIFDDLVSESHLGNLLEQVDEICSLITKLPFSFQDKEERFRFSPPYLVLIDWGHDERDYKAGRPDQAKRLSKKEWNRMMSHIRTIAERAWKQYGVRAVIHPHAGGYIEFEDEIQQLLKDIPYDIAGLCLDTGHLYYSKMDPEQWLRDYADRVDYIHFKDIDEHVYQQVMGEHIRFFDACAKGVMCPIGQGIIDYEAIYKLLKDIHYHGYITIEQERDPRNSDTSLRDVSQSLAYLKNVGY

SEQ ID NO: 163 - protein, 339 aa, Bacillus subtilis
  >ABP24567
MEKEVFSKMKTTIYDVAEKAGVSISTVSKVINHQPVGMKSKQKVLDAMQELNYKPSVLASALTGKRTSTIGFLLPDIANPLIAEMARRVEDRAHEYGFNVVICSTDFKSEKEERYVSLLRQKRVDGFILAGGFRNKQVIHELISDNIPVILLSESQPYSSLTTVTVDNFLGGYELTAYLISLGHSRIAVIAEDNASSRERIRGYSQALQESDLDIHEDLIVVTDSTAESAQSLASSLLQSSNPPTAMICCNDILAIGALLAAREEHVLVPEELSITGFDNTLISKSSDPPLTTVEVPVQSMCSQAVDLLIDEIEGKASEKQKILVLPKLIVRKSTSRFH

SEQ ID NO: 164 - protein, 41 aa, Bacillus subtilis
  >ABP24568
MSLVKNGDSIKVVFVFQKNEQIEEVELNSAQLSALLHSKQV

SEQ ID NO: 165 - protein, 52 aa, Bacillus subtilis
  >ABP24598
MDINDASEHLIQLKQDLIDRSKIEMINKLKRWAFSFLKHLNFEIQTFNYGFV

SEQ ID NO: 166 - protein, 111 aa, Bacillus subtilis
  >ABP24599
MKKRLIGFLVLVPALIMSGIILIEANKKAPVEVLESAWDEFGLFSFQIGKTDPSITIGMDHTKSEAKLREYLEHNLSREAKEKYKIYIFKDDIDKLEKEHREYLKANNPNK

SEQ ID NO: 167 - protein, 48 aa, Bacillus subtilis
  >ABP24600
MRFTAGGNLSTMDSQVLDVIKKAYNLGMVNKDNMLLRNEAINAYRNSI

SEQ ID NO: 168 - protein, 384 aa, Bacillus subtilis
  >ABP24601
MLPEYRKKTPEEILEEIERLKRGRLKVYIGSAPGVGKTYRMLQEAHELKAEGLDVVIGLIETHNRKETEDLIGDLEIVPKKNIDYKGRLLEEMDTEAIIKRAPDLVLIDELAHTNVPFSQRNKRYMDVEEILKSGINVLSAVNIQHLESLHDIVQQITGVQVRERIPDSFLHMAHEIILVDVTPEILRKRLSEGKIYHPSKIEQALNNFFTASNLGALRELSLREVANDVDERVEKANEKNGKNKPSGINEKIMVCVQHGSNAERLIRRGWRIANRLKTELIILHVTNEVSMKRSTENRKKIQDWKRLAIQFNARFIIEQIKKRHIAKAITDVAKEHDVTQIILGQSARSRWEEIRKGSIVNMIMRYTTGVDIHIVSDQQPRRK

SEQ ID NO: 169 - protein, 189 aa, Bacillus subtilis
  >ABP24602
MLKIIRLALLMIIICGILYPLLMTGLAQAIFPDQANGSILKNKDGQIVGSELIGQQFTKSNYFQGRISSIKYNAVGSGSNNYGPTNQEMLERTKSFIRVLEEGNPDLKTKELPIDLITNSGSGLDPDISVKAAKFQVNRVSNATGVSESTLNKLIDNTIDGRSLGIFGEPRVNVLKLNMKVQEIISKGN

SEQ ID NO: 170 - protein, 674 aa, Bacillus subtilis
  >ABP24603
MNKSNENSEMIKEAITQSFIKLNPLSMMKNPVMFVVEVGTFLVLLMLIMPSAFHSEEGYVYNLIVFLILLFTILFANFAEALAEGRGKAQADSLKKTKKDTVARRINKNGTVTDISSADLKKGDIVLVETGDFIPGDGEIIEGLASIDESAITGESAPVIKEAGGDFSSVTGGTKVVSDSIKVRITADPGESFLDKMISLVEGAKRQKTPNEIALTILLVTLTIIFLLVVVTLLPIANYVGVHIELSTLIALLVCLIPTTIGALLSAIGIAGMDRVTQFNVLAMSGKAVEVAGDINTIILDKTGTITFGNRLAAEFIPVSSTTQEELMQAAVITSLFDETPEGRSVLELAKNNGASWEASAYESAEIIPFTAEERMSGLIKDGHHYRKGAVDSIKAFVQEMGGPLPLDLQSKSEEVARQGGTPLAVSYNNRILGLIYLKDTVKPGMRERFDELRKMGIKTIMCTGDNPLTASTIAKEAGVDDFIAEAKPEDKIRVIREEQEKGKLVAMTGDGTNDAPALAQADVGLAMNSGTIAAKEAANMVDLDSDPTKIIEVVAIGKQLLMTRGSLTTFSIANDIAKYFAIIPAMFTVAIPGMQVLNIMRLHSPTTAILSALIFNAIIIPLLIPLAMKGVKYVPMSASKLLSRNILIYGLGGIVVPFIGIKLIDILVSVFMS

SEQ ID NO: 171 - protein, 389 aa, Bacillus subtilis
  >ABP24604
MKGHTRLLIPMSIILTIILVSLKVPQTLSPSIEVTTLEGVKQVISIGPVASLESIKHLGTNGGGFFGANSAHPFENPSPLTNVIEILSMWCIPASLTYTYGRFAKKQKQGWVIFGAMFILFIAFLSLIYVSESHGNPALTALGLDPSQGSMEGKEVRFGIAQSALFSSVTTAATTGTVNNMHDTLTPLGQITPLSLMMLNTVFGGDGVGLVNMLMYAIIGVFICGLMVGRTPEFLGRKIEPKEMKLITVALLAHPLIILAPTALAFLADIGKGSISNPGFHGVSQVLYEFASSAANNGSGFEGLADNTPFWNISTGLVMLVGRYISIIALLAVAGSLVQKQPVPETIGTFKTDNLLFIGILVGVVLIVGALTFFPVIALGPIAEYLSIR

SEQ ID NO: 172 - protein, 170 aa, Bacillus subtilis
  >ABP24605
MGILQIIVVIMLMLFMIKPLGTYIYHVFSNEPNKTDKIFNPIEKIIYKICGMKNRLSMTWKQYAGSLLLTNMVFIAVGYVILRFQYILPLNPNGIENMNSMLSFNTIISFMTNTNLQHYSGETGLSYFSQMAVIMMMMFTSAATGIAAAIAFIRGITSKGKTIGNFLKIL

SEQ ID NO: 173 - protein, 43 aa, Bacillus subtilis
  >ABP24606
MNNNLGGITLDDVCMLAVIAVIFAVFWAFVKWCDFTIGGGEKQ

SEQ ID NO: 174 - protein, 155 aa, Bacillus subtilis
  >ABP20078
MPKQQTAELKPFFHNKTVLVTGGTGSIGSQIVKRLLMLTPKQVIVFSKDDSKQYVMSQKYAEDKRLLFVLGDVRDHRRVNQVMKGVDIVFHAAALKQVPTCEDHPFEAIQTNLIGGQNVVEAALSHRVQHVINISTDKAVFKDTDYKLIKKKGLF

SEQ ID NO: 175 - protein, 56 aa, Bacillus subtilis
  >ABP20079
MPYEEYEELKKKTIKVIQRKNYSIRIIDQKFENDNLDQLYKEVARLLFERALKSSE

SEQ ID NO: 176 - protein, 196 aa, Bacillus subtilis
  >ABP20080
MGANNQGKVFEANIEKSAADQKLFFYRIKDVNPMFLKRGAAVSKNKYDCFLHFNGYLFPFELKSTKDKSIAFREKIIKPQQIKYLKEATQYPNIIPGFLFQFREPENKVYFVHIDEFLKYKNIAEKQLKHTYKNKVNKASIPIAICEEIGTEVRWMKKKVNYTYYLNKLCVELIKKEQSRDKPLHTYNTPVKTGVR

SEQ ID NO: 177 - protein, 93 aa, Bacillus subtilis
  >ABP20081
MYVLKSLLKEVYIVKKQWKPVDSRLNELMHEYSVSIEDLVERTGLPKQRINDYVSGFKSNMNIGTAMTFADAIGCSIEELYVWNFKERRQLIK

SEQ ID NO: 178 - protein, 43 aa, Bacillus subtilis
  >ABP20082
MKTVKEAIDEKDLQRAHRNLINLADNNEELMQEIRWIKKGTTL

SEQ ID NO: 179 - protein, 109 aa, Bacillus subtilis
  >ABP20083
MNLKNIDENRYKKTYSVQPNDIFFVVRKNGNQTPYLIYKDKNKMLKLINLQSGASNYCADTIDSLVGIYIKENQESPANKVNPIKEYFFAKSHETSIRVHNTFNYNPIK

SEQ ID NO: 180 - protein, 144 aa, Bacillus subtilis
  >ABP20084
MKTIKLYELVSEGKKPIIKFNDNVYEWIEESVDTMMMGKIIGASIEYEDSVRFLIDLNPFEAYNRSVARHDWRDDEGNCVLTWFDTSFYPKNGIEAIYLPINGRTEIAFDFTEEDSLLNEYAKVPQEISYVEWLENEVKQLISK

SEQ ID NO: 181 - protein, 51 aa, Bacillus subtilis
  >ABP20085
MIVTAWILLIMFGLFALSDLNLTEDETKHIKFFMLMKFFSVFIAAIAAGVI

SEQ ID NO: 182 - protein, 182 aa, Bacillus subtilis
  >ABP20086
MKNTEFKKTSFLEEYKRGDEMRRDFIIHEGYTAIEEIIKEVNQRGSLNEADIYYGTPKPQLSFSDVELGYMLTSMMEYATNHVGNPVDEECEFENKLAYFEYKDEIVQIFEVYGQGTESWFSKPSDDTIDKLNNTAYGVYLIQFDDFINYTKNKDSESEKLSPSSTILNDITGGYTVGRGSK

SEQ ID NO: 183 - protein, 49 aa, Bacillus subtilis
  >ABP20087
MLELDEYILKSEMDFADPEEIRSCIISFVSSLQQYIDLCKEELNEEYRV

SEQ ID NO: 184 - protein, 53 aa, Bacillus subtilis
  >ABP20088
MVELAKEENMLFFDHYPTEYGGWQTGNRDVWGIWGQRYLLKKVSDGCCEYVSR

SEQ ID NO: 185 - protein, 73 aa, Bacillus subtilis
  >ABP20089
MYGEDVEVTLDGNIKVKVFVFCLPTTCKEEKEKRALLTLKNLIDKRLKNEDLKYLDVQSDFVLIPKMIENGEF

SEQ ID NO: 186 - protein, 67 aa, Bacillus subtilis
  >ABP20090
MRVSSEALKIVIVQHLERDNDLMSEGKIIVLPCRDEKTAKEFEDFYRKKFPSTQLMSIEIVDSNIYG

SEQ ID NO: 187 - protein, 216 aa, Bacillus subtilis
  >ABP20091
METKKYVRIIRNASKYGDMTGQIFPLFGTWEDSYKIDGSDGVVYVRKKDVEVIVTENRRPKVDERVLITEVLLSSGHYKIGDIYTVLSVVDIYGTITVKEHSNCVISREYEVIVDEVKKEEADGMENVNQTVINNANTVFEKKDDKYFGYKSRFGDIVIGGAYSYRFVVQYAKTNQDVVVIPGDENTVTTPVCTTLEERLWQPEKAVKSSPRNLHY

SEQ ID NO: 188 - protein, 117 aa, Bacillus subtilis
  >ABP20092
MEVGDKIHNTNEQITALEKKKYQIETTLLEKQRDLLKLETQQNKEKLELLFELSEVLTQLQDEEWVSCMIALRIIRRNKRKYLNLFELVNEKAYINKDKFKVLHDEFFDLKQQLNEI

SEQ ID NO: 189 - protein, 66 aa, Bacillus subtilis
  >ABP20093
MIYKTFLPYADKVYLTIVDSAQREADSYFPMLDDRWKLTDKRHNKADEKNKYNYSFITFENNYRQK

SEQ ID NO: 190 - protein, 279 aa, Bacillus subtilis
  >ABP20094
MTQFDKQYNSIIKDIINNGISNEEFDVRTKWDSDGTPAHTLSVMSKQMRFDNSEVPILTTKKVAWKTAIKELLWIWQLKSNDVNDLNKMGVHIWDQWKQEDGTIGHAYGFQLGKKNRNLNGEKVDQVDYLLHQLKNNPSSRRHITMLWNPDELDAMALTPCVYETQWYVKHGKLHLEVRARSNDMALGNPFNVFQYNVLQRMIAQVTGYELGEYIFNIGDCHVYTRHIDNLKIQMEREQFEAPELWINPEVKDFYDFTIDDFKLINYKHGDKLFFEVAV

SEQ ID NO: 191 - protein, 40 aa, Bacillus subtilis
  >ABP20095
MFKVLDVLDGEKTKQNTYIYWLFVCGNFLFVVFYLADVFL

SEQ ID NO: 192 - protein, 101 aa, Bacillus subtilis
  >ABP20096
MLKDKNKITKSIEKINKLEEGLALFEEGDEEYLSVLVKIQGLYDEIADTALECFKEMTTKIRKTGQKRIGKGIDQLPYTIKENIADQVNELKGSFLDESKY

SEQ ID NO: 193 - protein, 72 aa, Bacillus subtilis
  >ABP20119
MDSYPESLKKETEEIKERVRNGNIKEDRIKEIAETTVEFLKSEEKRHKYFSEVAAAMADNLSEFFKSYLKGE

SEQ ID NO: 194 - protein, 503 aa, Bacillus subtilis
  >ABP20120
MKKLRVMSLFSGIGAFEAALRNIGVEYELVGFSEIDKYAIKSYCAIHNVDEQLNYGDVSKIDKKKLPEFDLLVGGSPCQSFSVAGYRKGFEDTRGTLFFQYIDTLKEKQPRYFVFENVKGLINHDKGNTLNIMAESFSEVGYRIDLELLNSKFFNVPQNRERIYIIGVREDLIENDEWVVEKGRNDVLSKGKKRLKELNIKSFNFKWSAQDIVGRRLREILEEYVDEKYYLSEEKTSKLIEQIEKPKEKDVVFVGGINVGKRWLNNGKTYSRNFKQGNRVYDSNGIATTLTSQSVGGLGGQTSLYKVEDPIMIGHIDLKGHDAIKRVYSPDGVSPTLTTMGGGHREPKIAVEYVGNINPSGKGMNDQVYNSNGLSPTLTTNKGEGVKISVPNPEIRPVLTPEREEKRQNGRRFKEDDEPAFTVNTIDRHGVAIGEYPKYRIRKLTPLECWRLQAFDEEDFEKALSVGISNSQLYKQAGNSITVTVLESIFKELIHTYVNEESE

SEQ ID NO: 195 - protein, 269 aa, Bacillus subtilis
  >ABP20121
MDINGKDLNKIHNIDCVQFMRENMGDCSIDLTVTSPPYDDLRKYNGYSFNFEATARELYRVTKDGGVVVWVIGDKTHNGSESGTSFKQALYFKEIGFNLHDTMIYEKDSISFPDKNRYYQIFEYMFVFSKGKPKTINLISDRKNKWYNGKKHIKGHYRKMDGEKVRHNKQNLLKEFGVRFNIWRIPNGHQKSTLDKVAFEHPAIFPERLAEDHILSWSNEGDIVLDPFMGSGTTAKMAALNNRKYIGTEISKEYCDIANERLRNYIGTI

SEQ ID NO: 196 - protein, 172 aa, Bacillus subtilis
  >ABP20122
MKKVIAIDMDQVLADLLSDWVAYINTHDDPFLKEEEILCWDIKKYTNTNNNVYRHLDYDLFRNLDVIEGSQRVVKELMKKYEVYVVTTATNHPESLKAKLEWLTEHFSFIPHSNVVLCGNKSIIKADIMIDDGIHNLESFEGMKILFDAPHNRNDNRFIRVMNWEEIERKLL

SEQ ID NO: 197 - protein, 165 aa, Bacillus subtilis
  >ABP20123
MALIILEGPDCCFKSTVAAKLSKAMKYPIIKGSSFELATSGNQKLFEHFNRLADEDSVIIDRFVYSNLVYAKKFKDYSILTEQQLRIIEDKIKLKAKVVYLHADPSVIKERLSIRGDEYIEGKDIDSILELYREVMSNAGLHTYSWDTGQWSSDEIAKDTIFLVE

SEQ ID NO: 198 - protein, 227 aa, Bacillus subtilis
  >ABP20226
MGYKLMAYGGYFLFCLFFLLMDGWRGMGICLIIAGLALLALEPYKIKAQKNIDKLKENAETLKHYESGFNPDNFFNTYKTKIAFKESDSLVKIYQLNRNEHIEEYTIPFSNIIESEITLDNQIISKVSKSGIVAGGLLAGGIGAALGGLSASSIQNEMVKSVTLKITVEDLGKPIHYIDFLPTQEVEGYNTQGYKKDSNIIQQALKNAEYWHGVMDVIIKKASKVAQ

SEQ ID NO: 199 - protein, 2296 aa, Bacillus subtilis
  >ABP20227
MSQNLKIILTPQADTSSKTVEQLNQQIKSLEKKLNSLKLNTNIDSTTLKALQEFSSAVDAYQKNLKSYNQTVRETSTVIKNADGSVEKLTQQYKKNGEILQRETKIINNRNTALKQETQEVNKLTQATEKLGQVQKKTVQRNLQGQPTKIVQKNRQGFDDIVYTTDPKTNSTSSKTTTNYDQQRRAIEQLKQDLEKLRQQGIVTDTTISSLGRKINTAQSAQQIEALQNRIRMLDDKSAAVAKNNELKKTIELYQRQAQVNVQNLNTRYGSSMGSSNRQAVQDYLNAVNSLNVSTGSNNIRSQIQSLNMQFRELASSAQAAANQASSFGAELTQTFKSMSTYLISGSLFYGAISGLKEMVSQAVEIDTLMTNIRRVMNEPDYKYNELLQESIDLGDTLSNKITDILQMTGDFGRMGFDESELSTLTKTAQVLQNVSDLTPDDTVNTLTAAMLNFNIAANDSISIADKLNEVDNNYAVTTLDLANSIRKAGSTASTFGVELNDLIGYTTAIASTTRESGNIVGNSLKTIFARIGNNQSSIKALDEIGISVKTASGEAKSASDLISEVAGKWDTLTDAQKQNTSIGVAGIYQLSRFNAMMNNFSIAQNAAKTAANSTGSAWSEQQKYADSLQARVNKLQNNFTEFAIAASDAFISDGLIEFTQAAGSLLNASTGVIKSVGFLPPLLAAVSTATLLLSKNTRTLATTLILGTRAMGQETLATAGLEAGMTRAAVASRVLKTALRGLLVSTLVGGAFAALGWALESLISSFAEAKKAKDDFEQSQQTNVEAITTNKDSTDKLIQQYKELQKVKESRSLTSDEEQEYLQVTQQLAQTFPSLVKGYDSQGNAILKTNKELEKAIENTKEYLALKKQETRDSAKKTFEDASKEIKKSKDELKQYKQIADYNDKGRPKWDLIADDDDYKVAADKAKQSMLKAQSDIESGNAKVKDSVLSIANAYSSIDISNTLKASISDVVNKLNLKDNLDPEELEKFSSSLGKLQEKMQKALDSGDEKAFDNAKKDIQSLLETYSKSDSSIDVFKMSFDKAQKNIKDGDKSLSSVKSEVGDLGETLAEAGNEAEDFGKKLKEALDANSVDDIKAAIKEMSDAMQFDSVQDALNGDIFNNTKDQVAPLNDLLEKMAEGKSISANEANTLIQKDKELAKAISIENGVVKINRDEVIKQRKVKLDAYNDMVTYSNKLMKTEVNNAIKTLNADTLRIDSLRKLRKERKLDMSEAELSDLEVKSINNVADAKKELKKLEEKMLQPGGYSNSQIEAMQSVKSALESYISASEEAASTQEMNKQALVEAGTSLENWTDQQEKANEETKTSMYVVDKYKEALEKVNAEIDKYNKQVNDYPKYSQKYRDAIKKEIKALQQKKKLMQEQAKLLKDQIKSGNIAQYGIVTTTSSPGGTSTSTGGSYSGKYSSYINSAASKYNVDPALIAAVIQQESGFNAKARSGVGAMGLMQLMPATAKSLGVNNAYDPYQNVMGGTKYLAQQLEKFGGNVEKALAAYNAGPGNVIKYGGIPPFKETQNYVKKIMANYSKSLSSATSSIASYYTNNSAFRVSSKYGQQESGLRSSPHKGTDFAAKAGTAIKSLQSGKVQIAGYSKTAGNWVVIKQDDGTVAKYMHMLNTPSVKTGQSVKAGQTIGKVGSTGNSTGNHLHLQIEQNGKTIDPEKYMQGIGTSISDASQAEAERQQGIAQAKSDLLSLQGDIDSVNDQIQELQYELVQSKLDEFDKRIGDFDIRIAKDESMANRYTSDSKEFRKYTSDQKKAVAEQAKIQQQKVNWIQKEIKTNKALNSAQRAQLQEELKQAKLDLISVQDQVRELQKQLVQSKVDETLKSIEKSSSKTQGKIKDVDNKISMTEEDEDKVKYYSKQIKLIQQQQKEAKKYIKQLEEQKKAAKGFPDIQEQITEEIENWKDKQKDFNLELYNTKKSIKDIYKSLADEVVSIYKEMYEKMRDIELEAHQKATQDKIDEIDKEDEEAKYQKELKEKNQAIQETKDKISKLSMDDSSEAKSQVKDLEKQLQEQQEALDEYIKDRSNTKRKEALQDQLDKDEESINNKYDDLVNDERAFKKLEDKLMDGKITDIAKQLNEFTKFINENMKSIGKSISNNLIDKLKDAASALNTVTTGNTTGKKVSSFASGGYTGTGLGAGKLAFLHDKELILNKTDTENMLEAVKQVRQTSTDNSVKTTSKWGQPGKISDVLSKSISLVTPAMNAAVASQTSLTKGLIPTLKNFSTPTVTPSTPQGNTSNNQNSFTINVTEASNAKETASLVYKQLANGLKNTGLNFNIT

SEQ ID NO: 200 - protein, 253 aa, Bacillus subtilis
  >ABP20228
MIRQSQYFLFDNEKSIDYGVENVNTESGLVEESFLGSRSVNETYVKGRSEPYTEGVKREAKQFPLNFYVGENYDEKKIRAIKRWLDVDDYKPLAFSENLDIVYYAMPVDTSDLVHNAARHGYVRLTMKCNSPYAYSRNTSTHSFDISSGMKTIELHNKGDVAIYPTVEILKIGDGDVKIENLSDYTDPFIFSNLKDREIVKVNGDKEIIESSLYGNERYDDFNDNYIRLDYGKNRLKVTGKCKLRLTFRFKYR

SEQ ID NO: 201 - protein, 880 aa, Bacillus subtilis
  >ABP20229
MITIRKDTEIKNIRLSLAKPDKTKIANIDEVLNPTVTLNHGSSVHELSFSIPLKATYDGVIKRNHVVDLLKPWYLIKTEFYGLAIWFIITKRTKSFSSEMDTVQVECRSLQHELSRISVLKYEETSKNLQEVVTDCLKNTSWTVGYIDTLFNVKRRQFDVSSTNKLDFLYSICEKFDAVPVFDTVKETVSFYKESDISKYKGLKLNPRQYMISMDDSDDADELVTRLYATGKDGISINSVNPTGQSYIDDFSYFLFPFQRDEQRNVISHSAYMPDELCHAILDYNDLVNSEGNAFNKLLTQKNEAETGLTELNNELYTLDLEVQKLLDRIEVAKKAGDDTSQLKAQLAVKQKAVALKKNQIATIESTISQISASISKLKEKLSFENNFSENQQKLLSRFISTTEWSNDSIYDENELYDDANEELESRNTPPVNVTLDIVNFFNCISEKHNWDRFSLGDIVRVQQSDLNTDIKAILSAITIDFEQSNISVTVTNGKRVQSDFEKVIKTVYRTNKISTELNKRKIEWDKVTENFNIRNDRISVQPAPPVIASDGTAITHKVNDNGSVDITIQWNYVDSNEDKYNIDGFEVYLHGSDDNEEYTFGSVQASENLQNVKYDRRTATFTGLPSNMYYTIGVQAYRRVDADIDINQILLSDIVKSNHPSENPYLPTPSIEVKGSLSGKVNGLYTISTESKPEEPETGTIWIDPKTNKQELFNGEEWIVSSAGSADSLNGFTASLTTSPNSIPVRDQSGVISGSIDGNAEMLGGRAASDYALTENIPVPPKFAKGVYTGDGTLSKQIPLAFTPDLVKITPISPEDSQLVIESQLGGYAYQVTSTGLSLIGGDLSYGALGNNLFITGSDSNCRGNKLNVKYIWEAYQQN

SEQ ID NO: 202 - protein, 285 aa, Bacillus subtilis
  >ABP20230
MGSLPTKLTEVIKLADFAELYNDPILSKKRIGSVEDPYLTYSETLTVYNGRALLTEIPNREFRVEVIGDKKEWREIEDGELEDNYFKVDYLMGVVFFNASNEGKSLTFNYSGEGASFFPASRIWIKRQGNMVIETLQGLIDDAEDTIIRMNERIAECERVTKRCIEITNWCRQATSDYEYVVENTRKIYLPMVYTYQDLMDTYPNPQIGWVVTIRDTGIEYRWDGFDWINISISDQFDGYNVVSSYIEPYNIRTVWLRTNSPPSKKRVKPSKDAPDGSMVWIRKG

SEQ ID NO: 203 - protein, 744 aa, Bacillus subtilis
  >ABP20231
MSDNLIPVNTMGYYDEETKQWVPIDAVALKSENYRFTADDISQKFNKIGDIDAIKATGNTLSEKIINEFNYRGINISWLGAKGDGTTDDSSVFSSIESTYQDKVFDLAGKTYVVNSFPNKNKYLNGYFIIDGNKYFSGYVSSFQTGNSNIIIGNNAAKNFRPGDQYKGIAGHNIIAIGENALSNASEYTKNTTAIGAGALFNNKYGVYNLAIGLQSQYYVTGVQGDAFKGTRNTSVGDNSMRFNKDGYSNVAMGRNALQTNEKSLWNTALGAAAMSGYAPLNLDSKTIINNSPQTAGYQVAVGTNSLYWSNGIGNVGVGVNAGREIKNSQRNVAMGYYAMSQLDSDVSFEGKQRFFPSIQAGYTWIGQDITLTHIGHTFIVGQNLSLALDGGEKFSTTVKSITVDTFTVSTTQIAQNEISGMAQVSEYYTTTGTYVWKDNNIQVSMGNHPFQNGYKVLMSVGGREAIYFTVANSTSSGFTVSTDIIGDESGAVKITEYSDTTPMAVNYDNTAIGVKAAWKMKKGSFNTAIGGLSLENNKGDYNTALGYMALKNNTTGNQNTALGYGALRFTTGGDEMKDISNSTGVGFNSRVSGSNQIQLGDGNSTPYSFNALQNRSDLRDKADIRDTVLGLDFINKVRPVDYKWDIRDEYVEIKEDGTVITHERDGSKKKNRYHHGVIAQEIQKVIEAEGIDFGGFQHHELSGGEDVMSIGYTEFIAPLIKAVQELSAKVEEQAKEIAALKKA

SEQ ID NO: 204 - protein, 355 aa, Bacillus subtilis
  >ABP20232
MTIQARQMLVSPGKYPIKGRYAMTAEYITFHNTANDASANNEISYMRNNNETVSYHFAVDDKEVVQGLPTNRSAFHCGDGEYGTGNRKSIGVEVCYSKSGGERYRKAEALAIKFIAQLLKERGWGVERVKKHQEWSGKYCPHRVLDEGRWNEVKAAIAAELKSLGGKSTTPTKTSTKPTTSSPSSSSAASGSLKSKVDGLRFYSKPSWEDKNVVGTVNKGIGFPTVVEKVKVGSAYQYKVKNSKGATYYITASDKYVDVTGSVKASSPTPKTTSTSSSSSSIKSVGKIKIVGVSSAAIVMDKPDRNSSKNIGTVKLGSTVSISGSVKGKNNSKGYWEVIYNGKRGYISGQFGSKI

SEQ ID NO: 205 - protein, 83 aa, Bacillus subtilis
  >ABP20233
MTKINWKVRLKKKTFLVAIFSATLLFVQAIASAFGYDLTVFGDNLTEKFNALLTFLTAMGIIVDPTTQGISDSEQAMDYDSPR

SEQ ID NO: 206 - protein, 379 aa, Bacillus subtilis
  >ABP20234
MLEQMISSSKVGVKINEWYKYIRLFSVPDSEILKAEVEEEIRHMKEDQDLFLYYSLMCFRHQLMLDYLEPKTLNEERPKVSDLLEKIESSQTDLKGILEYYFNFFRGMYEFEQYEYLNAISFYKQAERKLSLVADEIERAEFHYKVAEIYYHMKQTHMSMHHIVQAIDSYKAHENYTVRVIQCSFVIGLNYLDMDYPEKAIPHFKDALDKAREIDMSRLIGSSLYNLGLCSFAEEAYEKASEYFKEGIRVYQDNGYEHSNRILDILLMLTKTTFKMRNHSEGISWCAHGLSLSKNLNDEIMAKMFEFIHALYVDNDNEKLNSILNYLELKSMLSDVEDLASDAAKYYNEKEDHKVAVAYYEKVLYARKQIQRGDCLYET

SEQ ID NO: 207 - protein, 58 aa, Bacillus subtilis
  >ABP20235
MKLKHASVFILAIVLIGFVSTYLTNTQKDVQEARRGHTASIGFTDGHSYEIASRGHTS